European Patent Application EP 4 461 813 A2, published November 13, 2024. Title: COMPOSITIONS AND METHODS FOR INCREASING SHELF-LIFE OF BANANA. Applicant: Tropic Biosciences UK Limited. Application EP. The sequence listing filed with the application follows.

SEQUENCE LISTING (74 sequences)

SEQ ID NO: 1 - DNA, 1759 bp, Musa acuminata
  source 1..1759: mol_type = genomic DNA
tgcaatctctctgttgtgttctgtaggtataacttctcttgatctcttcttggcataccacgatggagcagaagctgctgtcgagaaaggctgcatgcaacagccacgggcaggattcgtcctacttcttggggtggcaggagttcgagaagaacccctacgatccaatcgccaacacaggagggatcattcagatgggtcttgcagaaaaccaggttggttatcccctctcatagcttctcctcattcgtcattcctgaaaccctagtgtttgattgatcccttaccgtcttgttcatcgtgcatgcctgcagctctcattcgatctcatcgagtcatggcttgaagaccaccctgacctcaccggattcaagaaagatggtggtttggtgttccgggagcttgctctgttccaggactatcatggcttgccagctttcaagaatgtaagcccatattatagcctcagctaatcgatccaggggaagattcgcatccattcttgatgtctctactgacctctgcaacacatacatttgcaggcattggctagatatatgggagaagtcagaggaaacaaagtaagtttcgagcccagcaagctcgtcctcacggctggtgccacttctgccaacgagactctcatgttctgtcttgccgaccctggagaagcgttccttctcccaactccgtactatccagggtactgcactgacctcgtcgatacctgagctatgttgttgggtcgccgtggtgacactcctttggatgcgcgtgacaggttcgacagggacctcaaatggcgaaccggcgtggagatcgttcccatccactgctcgagctcgaatggcttccgaatcacccgagcggcactggaggcggcactccgacgtgcgcagaagcgtagactgagagtgaaaggagtgctggtgaccaacccgtccaacccactggggacgacgctgacccgacaagaactggacaccctcgtcgacttcgccgttgccaatgacatccacctcatcagcgacgagatctactccggcaccaccttcggctcgccgggtttcgtcagcatcgccgaggccaccaagggcagggacgacgtctcccatcgcattcacatcgtgtgcagtctctccaaggatctcggcctccctggcttccgcgtcggcgcaatctattcggacaacgaggccgtcgtgtccgccgccaccaagatgtcgagcttcgggctgatctcttcgcagacgcagtacctcctggcggcgctgctatcagacaaggaattcaccgagacgtacgtccgcgagagccagaagcggctcaaagaacgccacgacatgctcgtggaagggctccggcgaatcgggatcggttgcttggagggcaacgcagggttgttctgctgggtggacatgaggcacctgctgaggtcgaacaccttcgaaggggagatggaactgtggaagaagatcgtgtatcgagtaggactcaacatctcgccgggttcttcctgccactgcgacgaaccagggtggtttcgcgtctgcttcgccaacatgtccgaggacaccctggagctcgccatgaggcggctcgagagcttcgtggattcctgccatcggcgccgcccaagacggcaattcttggccaaatgggtgctcggctcagcctcatcgtctgccgatcgcaagtccgagcgataacgcctgctaagctgccagtgactgcatgcatgatcactcctactacgatt

SEQ ID NO: 2 - DNA, 4242 bp, Musa acuminata
  source 1..4242: mol_type = genomic DNA
taggcggcacgcattcggcaactccaacccctacccctacctcaggataaacagcgcgcctctgcttgcctgggcccgtaagcgaagacgcggccgccgccgccgcccgccgacgacacgggtgggatccgtgtgctagaggaggaaggaccagacggaggaggacggtctcacgccagcgatcgataaaggcagccatgcgcgtcatagtccccctccaggccgtggtgcaggggaggggcggcctcgtcctcggttccctcatcccctgcgccctcttctacttcctccagttctacctccgccgcaaccgcccctcctcctcttccccgccgcccccttcctctgcctccggctccaacctgcccgagctcgcctccatccctcggtcgctctcgaggggcctcctctctccccggggctcctttggcccagcacgcctctcctcgcgcggcaccgccgtcgtcagggacgacgacaacccctactacgtcgggctgaagaggtgcgccgatgacccctacaatcgctcgatcaatccccagggcttccttctgcttgggctggcagagaatagggtgtgtgatcctcccttcctttgcttcctgctatgtcaatgggcgatatgaaagatttggtgcttgtttttggcacagttgtcattggatataattcaagattggttggtcaagaattggaaggagtcattgctgttggatgacgaggaggaagagttgagtatccagggactggcaacgtatcagccttatgatggatcgatggatttgaagacggtgagtgaaacttttctcccttttgttttctacatctttcgatctcatttcttggtgcacgctcttagagtctgtattgccactggttcagaataatatttgaataagatttatgatgcaaataccaacaggagaagcaatttagaacacctcagtatatgacctgtttatgattctttttcatgtccatcaattcagtccttgtcaagacttccttgttttgttattatgtgtagaaaaaaaaactagatacaaatttatgccctaatgtattgtgacatggcatctacggatggttgtgacgatattgtccttcttctccagcttagtcttggttttgtctgttcaattttgtgggccttttgcactgatgaagtctgcctgcctatttgttgtacaagaagctgattttgggtgtgtgcatgtttattcattttgatctatgttttttttctgatatttccatagatcaaaatgaagacaacatacttttgaaaatccctaagcgaagcatactttttattattataccaagagattgtacgcttaattatttgcttatatagatacttgattttatgactaaaaaggcagaacagcatcatggcaaaaggcaagagaagacaacattattaaagatccatcttggagacactttcactgatagatacattatgttgattcttgttttgtattatattttaccttttattaacctgatgatgcttaatgtgtggaattggatttaacaactcattcgtagttataaggcaatgtctataactgcatgttagatgcttcaaatctatttccaaattgacgtttcttattttgtcgcaatggatctttcataccttccatttcattagtttcataacagagaaaatactatgatcatatccacttctgatttttttaacacgataagaaaggttgaagtttttttgacgttagcttggaaataatggttcttgtattttacacttacaaattcaagcgagaattgcaaatttatatgtaactatgacatacaaattttaattaatttaccttgtattttaatttcaaatgtacttctggcatttggtggagcataattatggatttggtagtttgctgtgattaactggtgaatatatttgctacaagaatgaaaaaaccattgtcttcaggttactcactcaagatcttgtatgtccaaagttgctcatctttttatgtggaacatcaagtttgattacaaagctatgttgttctcacaaggttacatctagaattttcctctctggaaatcttgactataagtttggtggatactaagaactatagctgaaagaaaatcagccagcatgatcttcattgttcatctatcatttcatcttcaagaagtgtgatattatctcgtattatcaactgaaatattcttgtatttaggcttacatattgagatttaattgataattttgacttttttgagagacatttcctcccatggagaacatttgtgggataacttaataaaaatgcattccgtgcataacacatccttgtccattatggtgattcataggtttttctgcttctgcctaagtaatgggccatgctggttccttgcatgtggaatttgcttgagttattcactcacgtcttagataagtggcatccgttactaattccttcagtctactgagattttttcccaattctattccagtttgcaagagcaccactttgtctgatttcatttctgacttgaaatcattttttgtttttaattaggtgatgaattgctaatctgatttgttttatttactgtcatataaattcaaaagcacctgaatgttcttcattgctttttcaacaggctgttgctgaattcatgggtcaagtcatgcaggggtcagtttcattcaatccgtcacacgttgtattaactgcaggtgccactcctgctgttgagacactaggcttctgtctggctgaccctggagatgcttttcttgttccatcaccttattaccctgggtgactattagtttttactctaactgagtgatcaattttttatgagtcaagatagtatacaaaattaacaagcacccaatgcaggtgggacagggatatcaagtggcgaactggtgtagagcttattcctgttccatgccgaagcactgataactttagcataagtattgctgcccttgaactagcatacaaccaagtaaagaagcgaggcatgaaggttcgtgctgttcttgtttctaacccctccaatccagttggtagtcttatagatcgggagacactatgtggccttctggactttgttatggaaaaaaacatacatctgatttctgatgaaatatttgctggatcgacatatgggagcgataagtttgtaagtgtggccgaggttctagatgcagaaagctttgacaagagcagggtccatataatatatggactgtcaaaagaccttgctgttccaggctttagggttggagtcatctactcttacaatgaaaatgtcctggctgctgcatcaaagctggcaaggttttcatccatttcagctcctacccaacggttgcttatctcaatgctctcggatagaaaattcatctcagaatatcttgcagtgaacagagcgagactacatgacatgcatgccttatttgttgatggactgaaacagttgggtatcaagtgtgccagtagcagtggtggattctattgttgggcagacatgagcatgtttattcgaccatatagtgagaaaggggagcttaagctctgggataatctgctgaatgtggccaaggtcaatgtgacacctgggtcatcatgccactgtatcgaacctggatggttcagatgttgcttcacgacattgacagagaaagatgttcctacagttatggaaagaatacagaaaattaccaaaagcaattaagttactgatgtttcaaaactcacctcttcaggcatcacttttaataaattgaagtgacttcaaatgtttatgtagtgtgaggacgctgtagttcggcagtcagcatgtcatctctggacttcaacatgcaaccaaagttaggacaccgtcgcaagaatcaaacttggagaggtggagataaagggtggtgttgaaatactaaggacattattgaaatatacagtttgatgcgacttttaacctccacagctggctggtgcgacaatcttcttgctatgggtattagatgatagtttagaatcttctgtacctgttcacttcttgtttaagttgaattggcttttctagtagattgtgcatattctcctcattaagctgcagatgtagattcaagattttggtttctactggtaggatgggggatgttcattgacatataatcatttttggtcttgttatgacataatttagtttatgagtcatattgtttagttt

SEQ ID NO: 3 - DNA, 1876 bp, Musa acuminata
  source 1..1876: mol_type = genomic DNA
gtctctcaatctcttctcagcctaccagaatgaatcagatgctgctctccagaaaagctgcatgcaacatccatgggcaggactcctcctatttcctggggtggcaggagtacgagaagaacccctatgatccaatcactaacccgacagggatcattcagatgggtctcgcagagaaccaggttggttctctcactcagacaagttctcctcactcaagtcactcgtgacagtaactaatattaaggcctctcgttcatgcttgcagctctgctttgatctcatcgaatcgtggcttgagaaccatcccgacccagctgcattcaagaaagatggagcactactattccgggagctcgctttgttccaggactaccatggcttgccagccttcaagcgtgtaagtccataaacttaaactaatttaccggggatatatcagaaggatcacatccattctcgcatatatcaacagaatctgctgggttactaattgcagtccgcgatgcatacatctgcaggcattggctaaatacatgggagaagtaagaggaaacaaagtagctttcgatcccaacaggctcgtcctcacggctggtgctacttctgccaatgagactctcatgttttgtcttgccgaacctggagaagcattccttctgcctactccatactacccagggtacgtacacatccacaacagagccttgtcgaccaattactctacccatgcacgcgatcggttccatgtacttgaattgccatggtgacacactcacctttcccatgtgtgtctgacagattcgacagagacctcaaatggcgaaccggagcggagatcgttcccatccattgttcgagctctaacgacttcaggatcaccaaaccggccctggaagctgcataccaagatgcgcagaagcgtagcctcagagtgaaaggtgtgctggtgaccaacccgtccaacccattggggacgacgctgacccgacacgaactcgacattcttgtcgactttgtcgtctccaaggacatccatctcatcagtgacgagatctactcagggaccaacttcgactcgccggggttcatcagcattgcagaggccacaaaggacaggaacaacgtctcccatcggattcacatcgtgtgcagcctctctaaagatctcggcctcccaggttttcgtgtcggtgcaatctattcggagaatgaagcagtcgtgtctgctgctactaagatgtcaagctttgggatggtctcttctcaaacccagtacctcctcgcggcgttgctatccgacaaagaattcaccgataagtaccttctcgagaatcagaagagactcaaagagcggcacgacatgcttgtcgaaggactgcgcaggatcgggatcgggtgcttgaaaggaagtgcggccttgttctgctgggtggacatgagacacctgctgaagtccaacaccttcaaaggagagatggagctgtggaagaagatagtgtatcaggtgggactaaacatctcgccgggttcttcgtgccactgcgacgaaccggggtggttccgcgtctgcttcgctaacatgtccgaggacaccctaaccctcgctatgcagcggcttaaaagcttcgttgactccggcgattgcggcagtaaccatgactccggccatcagcgccccagaaagccattcttgaccaagtgggtcctccgcttgtcgtccaccgatcgcaagtccgagcgctgataacaccggattgctgcagcgaatgcacgatcgatcattctttacatttttacgccaaacagcatgtttcttttctcctcgtgtctttttgccttggatcacgcgatctgtctggttttttgagtgccc

SEQ ID NO: 4 - DNA, 3417 bp, Musa acuminata
  source 1..3417: mol_type = genomic DNA
ccgcaggcacccgtcggctagaggaagaaacaccaggaggaggagtagggttcgcctgccgctatgcgcgtcatagtcccgctccaggctgtggtgcaggggagaggtggcctcgtcctcggctccctcatcccctgcgccctcttctacttcctccagctctacatccgccgcgaccgccgctcctcctccgcctccaacctgcccgagctcgctcccatgcctcgttcgctctctaggagcctcctctcgccccgcggctcgtccgggcccgcgcgtctctcatcgcgcggtgcttccgtcgcccgggatgatgacaacccctactacgtcggccttaagaggtgcgccgaggatccttaccatcactcgtccaatccccgtggcttcatgcagctcgggttggccgagaattgggtgggtgttcttccttccctcagttttttactatttggatggccgatataaaaggatttggcctaccgtttggtgctcgtcttcggtacagttgtcgttggatatgatccgagattggttggtcggtaatgtaaaggagccattgctgttagatgaggaaggagagttgagtatccacggattggcgacgtatcagccttatgatggattgatggatttgaagatggtgagtaaaagttctctgctttcgttttctaggtcgattaatttcattaatcttgttaatactggtgcacattcttcaagtctgtgtttctaatagatttggcgaaattttcaatacggtttatgatgtaaaagctaatgggaaactgagcatggaaacataatagacgaccaccgatctcccttttgctgcccatcaatttggttctcatcaaatattcctctttttgttctttagtaaaactagatgcaaagttaagaaaatttgtatgcatttctttctttgtagtagtacaatgaatacacatattctgataaaaagttgatggcataacaaatgttgtgaattaatttcagaaatctgattcgtacgacaacatgttgccttatgaagcaaaacgtatctcatcagccatacccttccacgaattgaaagcttcttaaatccaattgtaggaccaaaccgaatgattaggcaatatctgtgcatgtctttctttgtagtagtataatgaatacacttcttctggtgaaaagatgatggcatggcacaacaaatgttgtgaattaatttcagaaatctgattcgtacgagaacatgttgtcttataaagcaaaacatatctcatcagccatatccttccacgaattgaaagcttcttaaatccaattgtaggagcaaaccaaatgattaggcaatgtcggtgcatgtctttctttgcagtagtataatgaatacacatctggtaaaaagatgatggcataacaaatgttgtgaattaatttcagaaatctgattcgtatgagaacatgttgtcttataaagcaaaacatatctcatcagccatatccttccatgaattgaaagcttcttaaagccaatcgtaggagcaaaccgaattattaagcaatatccatgtagatgattttttttatgttaacagacagatgttgcagaggtaactttaacacacttcacacagttgtgtcaaccttagaaagctgcatctagaattttatatttatagatgttaacaaatataggtgtattagacacctgcatgatctgcatttgcaatctgttattttattttcgagaattgtgaatgtttttgagttagtcttgttgtgaatgctataactttaagatttggatggcagattttacttgctgaaataactttctacccatgaagaatatctacaacataggccaaaaaaaatattcaagccatgcgtacatttcgttgcccattatgtgattttttatatttttgtatgactgcctttatacatatcacagctgatttcttgcttgtgaaatttgcttgagttattatcttaggtaagcgatcatacatgtctaattcgtaaatcactacccaagagttttctatatctattccagtttgcaagtggatcagtgtcttttgtcaaattttatatctggctatgatattttattattattattatttttcatgttaagagttgttaatctgatttttctttttaaaatctggcatataaatctaacatcatcttgagattgttcattgtttttcaacaggctgttgctgaatttatgggtcaagtcatgcagggatcagtttcattccatccatcacaaattgtgttaactgcaggtgctactcctgcagttgagacacttagtttctgtctggctgaccctggaaatgcatttcttgttccatcaccttattaccctgggtaattattattttatcctctaagaaaattttcattattacaagtaaacacgaaactaagaagcatccaatgcaggtgggatagggatatcaagtggcgaactgggatagaacttattcctgttccttgcagaagcactgataacttcagcataagcattgctgctcttgaactagcatacaaccaagcaaagaagcgaggtgtgaaagtttgtgctgttcttgtctctaacccctccaacccagttggtaatctaatagatcgggaaacactatatgatcttctggactttgttatggagaaaaacatacatctgatttcagacgaagtctttgctggatcaacatatgggaatgatagatttgtaagtgtggctgaagttctagattcagaaaacttcgataggagaagagttcatataatatatggactgtcaaaagatctttgtgttccaggctttaggatcggggtcatctactcttacaatgaaaatgtcctggctgctgcgtcaaagctggccaggttctcatccatttcgactcctacccaatgtttgcttatttcaattctctcgaatacaaaattcattacagaatatctcaaggtaaacaaggagcagttatgcgacatgcatgccttatttgttgatggactgaaacggttgggtatcaagtgtgctagcagcagtggtgggttctattgttgggcagacatgagtatgtttattcaatcatataatgagaaaggggagcttaagctgtgggataagctgttgaatgaagctaagattaatgtgacacctgggtcatcatgtcactgtattgaacctggatggtttagatgttgcttcacaacattgacaaagcaggatattcctatagttatggaaaggatccacagaattactgagagcaactaagttgttgaattttcagaattttcatcttcagcttgcattttttgataacttatgcaagtggctctctgtttgaagaagtgcattccaaaagtcggatggcaagaactaattcccattggcattca

SEQ ID NO: 5 - DNA, 1963 bp, Musa acuminata
  source 1..1963: mol_type = genomic DNA
ctctctctctttctctctctctctctctctctgtttgtgtgtgcgttcgtaatccctgttgggcagaatctctgtcttgttctgtacgtacatcatctcttcattgtataccacaatgaatcagaagctgctctctagaaaggcagcatgcaacgttcatgggcaggactcctcgtacttcctagggtggcaagagtacgagaagaacccctatgatccaatcacgaaccccggagggatgattcagatgggtcttgccgagaaccaggttggttctctctcgaacaagttctgcgctcatacacaaactaatcccatgcttaacgatctcgtcatgcatgcttgcagctctgctttgatcttatcgagtcgtggctgcacacccaccctgacgccgccggattcaagaaagacggcgcattaatattccgggagcttgctctgttccaggactaccatggcttacctgctttcaagagcgtaagtctataaacccaagcagatgaatcatggatatcatatcagaagaaatggtttgatttcttatcgatccctgcattgcgtacttccgcaggcattggcaaaattcatgggagaagtacgaggaaacagagtaactttcgagccctgcaagctcgtcctgactgctggtgccacttctgccaacgagacactcatgttctgccttgccgagcccggagaagctttccttctgcccactccatactatccagggtatgcatcgacagcaaaacctcgacgacgactactactactactcttggcatgcacgcattgctcaaacttgtgtgtgacagattcgacagggacctcaaatggcgaaccggagctgagatcgttcccatccactgctccagctccaatggcttccgagtcaccaaagtggccctcgaagcagcgcaccgacacgcgcagaagcgtggcctcagggtgaagggagtcctcgtgaccaacccttccaacccattgggcacaaccatgacccggcaagaactggacaccctcatcgacttcgtcgttgccaaagacatccatctcatcagcgacgagatctactcgggcaccagcttcgactcgccggaattcgtcagcatcgccgaggccatcaaggacagggacgacgtcgcccaccgcgtccacatcgtgtgtagcctctccaagggtctcggtctcccgggattccgcgtcggtgcaatctactcaggcaacgacgcggtggtgtctgccgctacgaagatgtccagcttcggtctgatatcttctcagactcagtacctcctcgcagcgttgctctccgacgatgagttcaccaagaagtacattctcgagaaccggaggaggattaaagaacggcacgccctgctcgtgcaagggcttcgtaggatcgggatcagatgcttagagagcaacgcgggtctgttctgctgggtggacatgagacacctgctcaagtccgacaccttcaaaggagagatggagctgtggaggaagatagtgtatcaagtgggactaaacatctcgccgggctcttcgtgccactgcgacgaaccggggtggttccgcgtctgcttcgccaacatgtcggaggacacactcaacctctccatgcaacggctcaagaacttcgtggactccggcgagcatcgcaggacccacgattctggccatcggagtccgagaaggcaattcttgactgcatgactattcctacaattcttatagtttgtatatcccaagaagaagtagataacgaagaagtagaagaagaagaagacattatttaatttgtgagggtgttttttccctggatcaccacaatctgcttggatttttggtggccatggtctcatcatctataagatggtttgtatgtttagctcctcacttcctcaagtctgtattcggaggacagaatggactaaagcaacatcatttgtgcaag

SEQ ID NO: 6 - DNA, 1653 bp, Musa acuminata
  source 1..1653: mol_type = genomic DNA
atgccgcagcagctgctctccaggaaggccgcgtgcaacacccatggacaggactcctcctacttcctgggatggcaggagtacgagaagaacccttacgatcccaagacgaaccccaccggcatcattcagatgggtctcgcagagaaccaggtctgataatggtcatgaatcccatttccgcattctcggcatgctcgctgatagccaccgagtcttgatcttcatgtcacgtttcatgcagctctccttcgacctgatcgagtcgtggctcgaaagccaccccgacgctacggggctcaggcgagacggcgtcctcgtgttccgcgagctgggccttttccaggattatcatggcctgcctgagttcaagaaggtaagcattggataccgtctctattctcaaatgtgagggaatgagcgatcttccctgtgttgatcgatccgcttctacgtaaacgttcgcaggcactggcggatttcatgggagagtcgagacgaaacacagtgaaattcgatccccacaagctcgtcctcacggcaggcgccacttctgcaaacgagactctcatattttgcctcgccgaacccggcgaagcattccttctccctactccatactacccggggtatggaactagggacctgccaccctttccattctcatacctacactgtacattagtctcacacaactacgtgcataacagcttcgacagggatctcaaatggcgaactggtgcagaaatcgttcctgtacgttgttcaagctccaatggcttccggatcactaaggcggcgctcgagaaagcccatcgacgggcacgaaagcttcacttgagagtaaaaggagttctgatgaccaacccttccaatccattgggcacgacgatgacacaggtcgagctcgacaccctgatcgacttcgtcgtcgccaaagacatccatctcatcagcgacgaggtctactcgggcaccaacttcgactctccgggggtcatcagcgtcatggaggccatccagggccggaaaaatgtggcacatcgcgttcacctcgtctacagtctctccaaggatctcggcctccctgggttccgagtcggtgcaatctactctaataatgagacggtggtggctgcggccactaagatgtctagctttgggctcgtctcttcccagactcagtacctcctctccgcactgctctcagacaaggagttcagaagaagctacatcgtggagaaccagaggaggatcaaagagcggcatgacctgctcgttcgtggactcgagaaaaccggcatcaattgcctgaatagcaatgcgggtttgttctgctgggtggacatgagacacctgctgaagtccaacacctttgaaggagagatggagctgtggaagacgatggtgtaccaggtggggctaaacatctccccgggctcctcctgccactgcgacgagccggggtggttccgcgtctgcttcgccaacatgtcggcggagacgctcgagctggcgatccaacggctcgacgatttcgtagtttcctgtcatggccacaaggtgatctgcaactcaggatgcaggatgcaatcatgcatgcccaaatggatccttactctgccatcctcggatcgcatgttggagagatga

SEQ ID NO: 7 - DNA, 1662 bp, Musa acuminata
  source 1..1662: mol_type = genomic DNA
atggcccagatgctactctccatgaaggctgcgtgcaacactcatgggcaggactcctcgtacttcctggggttgcaggagtatgagaacgacccgtatgatccgaagaccaaccccaccgggatcattcagatgggcctggcggagaaccaggttcgcattccgtggatcgccatcatcttttgccggctctctctctctctctctcgcttactcttaccctgtcgatcgtgcagctctctttcgatctcatcgagtcgtggctgcagcgacaccccgacgcggcggggctaagaagagacggccgcgtcgtgttccgagagctggctctcttccaggattaccatggcttacctgagttcaagagagtaagtgctgggttcgaacagatagagagggatgtcgcgcttctcttttgccgcatggtaatgcgatgcgtgcgcttctttgagatcccgtcttcacgttctgcacaacgtacgtctgcaggcactggcggatctcatgggcgatttaagaggcaacaagatcgagatcgatccgcgaaagcttgtcctgaccgccggagccacctctgctaacgagattctcatgttctgtctcgccgaacccggcgaggcctttcttattcctactccatactatccagggtaaacacatcatctctcccactgttcataaacctcagtaactccgcgactaacatccgctaaacacaggtttgacagggatctgaaatggcgtaccggcgcggagatcgttcctgtacactgttccagctccaatgggttccgaatcaccagagccgccctcgaaaaagcctatcaaggagcgcgaaagcgtaatctgatagtaaaaggagttctgatcaccaatccttccaatccattgggcacgacgatgagtcggaacgagatcgacgccctcgtcgacttcgtcgtcgccaaggacgtccatctcatcagcgacgagatctactccggaacgaccttcgactcgcccgggttcgtcagcgtcacggaggctatcgagggcagagcacacgtaacggatcgcgttcacgttgtatacagcctctccaaggatctcggcctccctggcttccgggtgggtgcaatctactccaacaacgaggccgtggtggccgcagctaccaagatgtcgagcttcggcctcgtctcttcccaaacccagtacctcctctcggctctgctctccgacgaggagttcagaggcaattacaccggggagaaccagaagaggatcaagcagcggcacgaccggctcgtccaaggccttgggcggagtggcatcagctgcttaaagagcaatgcgggtctgttctgctgggtggacatgaggcacttgctgcgttccaacacattggagggggagatggagctgtggaggaagatagtgtacgaagtggggctcaacatctcgccgggctcctcctgccactgcgacgagcccgggtggttccgcgtctgctttgccaacatgtcggtcgagacactcgacgtcgccatgcggcggctgcaggacttcgtggcctccggccgagcccacgacgacggcagccaccaaaggaagaagccaatcttgggcaagtggatgctcaccttgtcatcctcggaccacaggtcggagaggggatggtaa

SEQ ID NO: 8 - DNA, 1884 bp, Musa acuminata
  source 1..1884: mol_type = genomic DNA
atggggattcccggtgacgagatcctctccagggtcgctacgggcgatggccacggtgagaacacctcgtacttcgatggctggaaggcctacgataatgatcctttccacccgattcataatcccaatggtgtcatccaaatgggactcgcagaaaaccaggtaatgcttgtttctggctctgtccattactttctcctcctcctgctgctgctgctgctaatgggtttcggtctgcctttcctcagctctgcttggacttgatgcgagattggatcaggaagaatccacaggcttctatatgcaccaaggagggcgtttcagagttcgaagccatcgctaacttccaggactaccatggcctgccggacttccgtaaggtaatcaccgtctgcagccataatgcagctcctcgatcccttactcatgcgtgccatgaacgatgagggcacagttggatcgatatgcgttgctatagccgaaaggtaatgacgcgatcatctatggaaatgcacaggccattgccaagttcatggagaaagcgagaggaggacgagccaggttcgacccggagcgcatagtgatgagcggtggagccaccggagctcaagaaacgatcgcattttgtctggccaatcccggggacgccttcctcattccgacgccatactacccagcgtacgtatgcctgttgagtcaacattctgatctctcaagtaattgcgtcgtcaacttccccgttcgaacaaatgttccagccgaccaatcagtcgtgcaatgacccaaacgacagtcaaacttttatctgcctgagcattgaccaaaaccacaccattcaacgtaattgtggtcatgcaatccgacactaaagaacgacatttggttcttctcaggttcgatcgagacttcaggtggagaactggagttcagctcctccctattcgctgccacagtcacgacaacttcaagatcaccgaagccgagcttgctgctgcctaccggaaggcgcgcgactctaagatcagggttaaaggaatactaataaccaacccgtcgaatcctctgggcacaaccatggacagggagacgctaagaaccctagtaagattcgcgaacgaggaaaggatccacctagtctgcgacgagatcttctccggcacagtcttcgacgggccggaatatgtcagtgtggcggagatattgcaagaggatccgtcgacctgcgacggagacctaatccacatcgtctacagcctgtcgaaggacctcggcgtccccggattccgtgtcggcatcatatactcgttcaacgacgcggtggtcagctgcgctcggaggatgtccagcttcggactggtctcgacgcagactcaacgcctgcttgcttccatgctgggagacgacgacttcaccaccgacctcttggcggagagcaggaggagattaatgcacaggcacaggacgtttactgccggcctcgaaggcgtcggcattcgttgcttacagagcaacgccggactattctgctggatgagcttgaagcctctgctgaaagacgccacggcggagggcgaggtcgagctgtggcgggtgatagtgaacgaggtgaagctcaacatctctccggggtcctcgttccactgcaccgagccggggtggttcagggcgtgctttgccaacatggacgaggagaccatggagacggccctgcggcggatcaggacgttcgtgcgccgggcgaacgacgcagctactgccgccaagaccaagaagaggtgggacacatcgcttcgcctgagcttgccacgaaggttcgaggagatgaccgtcctgacaccgcgtctgatgtctcctcgctctccgctcgttcaggccgccacctga

SEQ ID NO: 9 - DNA, 2504 bp, Musa acuminata
  source 1..2504: mol_type = genomic DNA
gcagcagctgcttctccttcttctctgctcgcttcagccttttccggtacgtacctgagataacgggtcacatgaggatctacggcgaggagcacccaaatcagcagatcctctctcggatcgcgaccaacgacggccatggcgagaactcctcctacttcgatgggtggaaggcctacgagaaggatcctttccacctcaccgacaaccccacgggggtcatccaaatgggactcgcagaaaaccaggttagagttccttcatggtgatgattaatcgcacatgccttccgtcaattgccactccctgcggttgctaatctaatctgtatgtgggttttgggtctttctttcctcagctttccctcgacttgatccgagactggatgaagaagaacccgcaggcttcgatctgcaccgaagaaggggtctcagagttcaaagcaattgccaactttcaggactatcatggcctcccagccttccgaaaggtaatgatttcaacccaaaacgcagcgctgcagctgcttgtcctcactgtccaagtagctacatacgtccaatatgataaagctgggactgacagccacttacggcccgagccctgcctgctcaccctggataagggataagctaatgatggtgtgatttgctgacacgcgcaggccatcgcccagttcatggagaaggtgagagggggacgagccagatttgacccagaccgcatcgtgatgagcggtggagccaccggtgctcaggaaaccatcgccttttgcctggctgatcctggcgaggccttcttgattccaacgccatattatccggggtaagtgttcaggtgtactaatctaccgagttctttatccggcagaggatctaatggcatctgcatggtttccagattcgatcgagacttcaggtggaggacaggagttcagctcctccccattcactgccacagttccaacaagttcaagatcacccaagccgcactggagactgcttacaggaaggctcgaaactcacacattagagtcaaaggaatactggtgaccaacccatcgaaccctctgggcacaaccatggacagagagacgctgagaaccctagtcagcttcgtcaacgagaaaaggatgcacttggtgtgcgacgagatcttctccggaaccgtcttcgacaagccgagttacgtgagcgtctccgaggtgatcgaagacgatccctactgcgacagggatctgattcacatcgcctacagcctctccaaggacctgggcgtccctggcttccgcgtcggcgtcatatactcctacaacgacgccgtggtcagctgcgcgaggaagatgtcgagctttggactggtctcgtcgcagacgcagcacctgctcgcttccatgttgggagacgaggagttcaccacgagtttcttagcgacgagccggacgaggttgtgcgggcggcgcagggtctttacggacggcctcaagcgagtcgggattcattgcttggacggcaacgcggggctgttctgctggatggacttgaggccgttgctgaaggaagcgacggtggaggcggagctccggctgtggcgggtgatcatcaacgacgtgaagctcaacatctcgccggggtcgtccttccactgctcggagccggggtggttcagggtatgcttcgccaacatggacgacacggccatgaagatagcgctgaggaggatcgagagtttcgtgtaccgggagaacgacgccgctgtgcaggcgaagaacaagaggaggtgggacgaagcgctgcggctgagcttgcctcgtcggaggttcgaggatccgaccatcatgacaccacatctgatgtctccccactcgcctctcgttcaagccgccacctgaaacatcgacagcggcgtgtctgatgtcaacgaaggttaattaccgtctgatatgttgcacatttctttgttctttggattatttatttttttttttttgggaaaaatgggttgaatgttcccactaagttatattagattgttgttcggtctcattcatgttataggaaacgaggatagaattgcttgcctctctctttcttttatatatggaaatatgttacaattggcctaagcttatttgatgacattaatttcacaagacaaagccttctaattaatgtttcggaccaaatgcaggagctcactacatacatttgttacacttcatatgttcaaaattagtccagtttaccggtgactcagttttaaaggttataaatggttctgattcaagtacttatctttggttctgttaattggttcaaaccgaatcgattttaatttaaacaatattaatttaattaaattttttaattggtttaaatcgattaatcaaatcagttgatcagggaaaatattattgatgtcttactcaactcgatatggtctatactcacgtgcgtaggaatgtccgagatgtctctgagataaaaacatcgtgctttcgtgat

SEQ ID NO: 10 - DNA, 1584 bp, Musa acuminata
  source 1..1584: mol_type = genomic DNA
atggttaagggtgctgagtcctgtgtgccactctcagaagtggcaacttccaacacccacggggaggactccccttactttgctggctggaaagcttatgatgaagacccttatgatgctgcaagcaaccctgcaggggtcattcagatgggtttggcagagaaccaagtaagctattactgatgcatactcattttagcataagaagaagttgtcttcatttctcttgcctgactgtgcccttgtggcctttctcaggtttcatttgatctactggagaagtatttagaccagcacccgggagcatccggctggggatgtggtatctccggcttcagagaaaacgctttgtttcaagattaccatggtctacaaacttttagacaggcaataagcataacctgggaacgatcgtgttgcttatccgttcgtaattgtttcagagaatcacgctcgactacaactgtgtctgcaggaaatggcaacttttatggaacagataagagaaggcagggcaaagtttgatcccgaacgcatcgtcctcaccgcaggtgcaaccgccgcaaacgagctactcaccttcatcttagcagatcccggagattgtttgctgatcccaacaccttattatcctgggtaagagctacggccacctcacagtgctgccgcttgttaatcttggcttaattaggttaacaggaaaaccacttctaatccaggtttgacagagatctaagatggagaactggtgttcgtatcattccggtccactgtagcagctcaaatggattccaagtaactctccaggccttagaagatgcgtacgtgaaagcagaaggcatgaagattagagtcagaggacttctcctcacaaacccatcgaacccgttgggcaccgcgatcgcaaggcatgtactcgaggaggtattagactttgtgacgcagaaggacatccacttgatctcagacgagatctactcaggctccgtgttctcctccgatgagttcgtcagcgtcgcggagattgtcgaagctcgcggctacaaagattgtgaccgagtccacatcgtgtatagcctctccaaggatcttggcctgcctggatttagagtgggagcaatttactcgtacaacgatagagtggtgacgactgctaggaggatgtccagcttcacattagtctcgtctcagactcagaggatgttggcttcgatgctggctgatagagggttcactgagaactacctgaagacaaatagagaaaggctcaagaataggcgtgatttcatcaccgaaggtctcaagaatgccgggatcgagtgcttgccagggaatgctgggctcttctgctggatgaatctggcaccattactcgaagagcccaccagggaaggagagctgagactttggagcttgatagtgcacgaggcgaagcttaacatatccccaggctcttcctgccactgttcggaagcaggctggtttagggtatgctttgctaatatgagccagcaaacactggaagttgcagtgaggagaataaaggacttcatgaagaacatgaaggcaatacaagagaaataa

SEQ ID NO: 11 - DNA, 1675 bp, Musa acuminata
  source 1..1675: mol_type = genomic DNA
atgcctcagatgcttctctctaggaaggctgcgtgcaacacccatggacaggactcctcttacttcctggggtggcaggagtacgagaagaacccgtatgatccacggacaaaccccaccggcatcattcagatgggtcttgcagagaaccaggttggtacaccatggacgacacctcctcctgcttcgtcttcttcttctctcccactgtacccacctgctaatgctattgttctgtgcagctctctttcgatctcatcgagtcgtggctggagcgccaccccgacgccgcggggctcaggcgagacggcgctctcgtcttccgggagctggctcttttccaggactatcatggcctgcctgctttcaagaaagtaagttgtactcggcttaagctactcttacatcgctttctcttgcgcatgtcaatgctgactttgctacgcgaacatgtgcaggctctggcagatttcatgggagagttaagaggagacaaggtcaagttcgaaccgcacaagctcgtcctcaccgcaggctccacttctgctaacgagactctgatgttctgcttggcggagcccggtgaagcgtttcttctccccactccatactatccagggtatatttccgtcaccatcacacactgttcgtcgaccttgtctacgtaaattcagtgcctgggtgacgtcgttaacattactgcacgtaaatctttgacaggtttgacagggatcttaaatggcgaactggcgcggagatcgttcccatccactgttcgagctccaatggcttccgggtcaccaaggccgccctcgaaaaagcctatcaaggagcgcgaaagcgtaatctgagggtgaaaggagttctggtcaccaatccttccaatccattgggcacgacgatgactcggtgcgagctcgacaccctcatcgacttcgtcgtcgccaaggacatccatcttatcagcgacgagatctactccgggaccagcttcgacgcgcccgggttcgtcagcgtcatggaggccatcgagggcagacaacacgtctcgcatcgtattcacgtcgtgtacagcctctccaaggatctcggcctccctggcttccgggtgggtgcaatctactccaacaacgaggcagtagtggccgccgctaccaagatgtcgagctttggactcgtctcctcccagactcagtacctcctctcggttctgctctccgacaaggagttcaccagaaactacattgaggagaaccagaagaggatcaaggagcggcacgaccggctcgtccaagggctccggagaagcggcatcagctgcctgcagagcaacgcaggtctgttctgctgggtggacatgaggcacctgctgaactccaacacgttcgaaggagagatggagctgtggaagaagatcgtgtaccaagtggggctcaacatctcgccgggctcctcctgccactccgacgagcccgggtggttccgcgtctgcttcgccaacatgtcggcggccacgctcgacctctcgatgcaacggctgcaggatttcgtggcctcccgcggaggccccaatgacggcgcctccgggccccggcggcaaaggaagaagccaagcttgggcaagtggatccttactctgtcgtcctcagatcgcatctcagacagaggatgttag

SEQ ID NO: 12 - DNA, 4149 bp, Musa acuminata
  source 1..4149: mol_type = genomic DNA
agaattgttataaaagagtgtggccaacggcgacgcttccttctatgtttccaaatacaatgcaaaccaacaaggtataaaataatctcgctcctcttcctcccgtcgatgagcccaaccccctccaagaaatccgccgacgccgccgcagccgcagccacagcgacccaagcccggtcgtccgcaaccggcctcggcggtggagggggcggcgcgggcatgcggctcatcgtacctcttcagggcgtcgtccagggccgcggcggcctcgtcctcggcaccctcatcccctgcgccctcttctacttcctccagttctacctcaggcgcaaccgctctcctcctcctacttcgccgcaaccccccgctgccaacggccccgatctccccggcatcgtccggtcctcctcccgcaacttcctctccgcccgcggctcctccggccacgccgccgtctcctcccgcgcggcctcgatcgccagatccggcgattcgccttacttcgtcgggactaagaagtgctccgaggacccttaccatcccgtcgataaccccgacggcgtcatacagcttgggttggccgagaaccgcgtagctttcttttaccctagaaaaactgtcatctttcttcttccttttggggttttatacccgtgaggagtttcttatcgattgttgttggtttgctgcagttgtctttggatctaattggggactggcttgcgagaaatgtgacggataccctactcgacgagcggcagggtgggctgagcatcagcggattggcgacgtaccagccttttgatgggttggtggaattgaagatggtgagcaatcgacctcctttcaccgcacaactagtttagttgtttcttttcctatgaatagcaattagttttcctgttgtttctcctcctgcttcacgctcgaactttctgtagtaaaaccagaattttcttttctttattgcttcacaacttctgcggtcccatcagtagtcatgttagtctgatttaaatcactttgctctgctggtcaatatgaaagttcagatcttttcatagatttttagattattacaggttgatgttcaagtaatgcttaacttatgttctaagatttcttttttttttttttttagtcagaatgaaaacttttagttttcctgcaagttcaccttccttttaagctgcaagttccgtggatatttttttatgcatgaacacataagacgtctccaaattttaatcaactcagtgagggggacaaaagagtttgccattcatctttgccaattttcaaacttttgctaaagttaagtggtttcatccaaggaggagtcatctttttctattagaggaattcacctgaaagttccttcttgccatcttgcaaaacatttggtggaaataagttaaatcttacggagagaggaagaaaaagacattattttcttttgtaaaacataagaaaaaagagcctgtgccctaaagttctttccttgtaaggaagaatgggttgggggaataaagagaaatacatggaaagagaagtcacttctccaagcaatattaataccaagtggaaatcaactctgttttcacaaaaggttttcatatcttcggcgtgaaggagggtgtctttggaaacacttctgggaaatgagttgatatttatgaaactacctatattgtgtaatcaaagtcggaaagtcgaactcagaagtaaagcctttattcacttttgagactcaactatgcataccgaataccaaaacaacaaattctacaaatttctttatggatgtctttttttccgtaagtattaaaaccatgagcagtcgatagggtgcatgattcttaaagaatttagctttctggattaccggagttggtgctttactaggttatcatgtgtcggtttctactgaagaagttacataaaggtcataaatgtagcttggctggtcaataaggtatctgcaattattacgagatttttttgtaggttttgcaaatatctggcaaaggttttttcataatattaccagctgcagctatcatatttggtttgtcgatgatgcctcaatgttgtgatgattatcccatattgcttttactatcttcttttgttgtttcaggatgcataactaagtttaagaaacattttatttcaccctaaaagatgtggttatgatatgcatcgattaacagacagtcaggctgatggttgtcttctgaagcatgtattcaattatatcattgtaattagcgttccagtacacactggtggtggattctttgctcatccattccccttctggacatgctgtgtgttcttctctttagccatgttttatatgattgggctattttaattgccgggatatctaatgaagcaataataactgagagaaagaaaaatatcttggaaatgttacgtgtaagcattcatttcgaaaaggcaggtgatcttggcgtactgcttatgtttgttgaatatgattatttagacttctctctgttttatcgtcttactagacctaattgtatgttctttataggattgatcttggaaagattttgtaatatcatactcatgtttacttttgataggctgtggctgaatttatgggacaagtcatgcaagggtcagtctcgtttgatccatcgcaaataataatgacagctggtgcaactccagcaattgaaattctcagtttctgcctggcagatgctggaaatgcatttcttgttccttcaccgtattacccagggtgacttgcttgttccaccaaaaacttgtctccatgtttcatactgagacatttttacaattttagtattttgacgtacaggtacgacaggaatataagatggcgagctggcatagagttgatacctgttccatgtcgaagcactgacaactttggtttaagtattcctgcactcgaaagagcatacaatcaggcaaaaatgcgaggtgtcaaagtgcgagctgttcttttctcaaacccctccaaccctgtgggcaatcttctgcacagggaaacattacgagaccttcttgactttgttacggagaagggcattcatgtcattgctgatgaagtgttcgcagggtcaacccatggtactgaggattttgtgagcatggcggaagttttaaacacagatgagtttgatagaagcagggttcacatagtatatggcttgtcaaaagatctctccgtcccaggctttcggatcggtctcatctactcttttaacgaacatgtcattgcggctgcctcgaagctggcaaggttttcctccgtttctgttccaacccagcacttgctcatctcgatgcttaatgacactaagttcatcacacaatatatcaagacgaacagagagagactccgagtaatgtatgcattgttagtgaatggccttaaacagttaggtgttgagagtgtcaaaagcagtggtggtttttactgttggacggatatgagcaaatttatgaaatcatacagtgagaaaggggagcttgagctatggaaggagatgcttaatgtagctaagattcatttgacacctggaacggcatgccattgcattgaacctggatggtttcgtttatgcttcacaacattgactgagaaggatgtgcctgtagttttggaacgcatcaagagagttgttgataaccattgagtctactaaagcagaaaggtagaggtctttggtacaaatatgttcataaggctggaaagtcgatcacatcgagtctctttcagtagtctcgtatcctctccagggttgtcatcaattttggtagtgtaggcttcgcttcatgcttctcttctccttgctgatgtaactacatcaaggtgcaccactactcgtgcagagacctccgcttggtgaagagatttcttttcacttaccagttgctaatatatgctctcatcttgttaccatttgcaatgaacggaaagcatgtaagcaccctcttctttaggtaatcctgtgatggacaaattggtttagaatgtgagtataatttccatatctttcattacttgtctattaagtcagtaatgtggaagtaaagaagaggtttttaatccgatgcttgtaatggtagacaggtttattagcc

SEQ ID NO: 13 - DNA, 2294 bp, Musa acuminata
  source 1..2294: mol_type = genomic DNA
tagctcgtgttctcccttctccccaggcttcccagtactcgcctaagatcgtaacgtcggcaatggggctccacgttgatgaacactcaaattacaatgtcctctccagcatcgcaacgagcgatggccacggggagaactcctcatacttcgatggctggaaggcctacgataatgatcctttccaccccatcgacaatcctcagggggtcatccaaatgggacttgcagaaaaccaggtaaatgctgtttcacaactagttcggtaattatggtagttttttcatggcctatggccaaaaatatgccttccgtattctcctactacttggaatgctaacgggtgctgcgttttccttatctcagctctgcctggacttgatgcagcagtggatcaagcagaacccacaggcttccatttgcaccggcgagggcgtttccgagtttaaggacgtcgcgaacttccaagactaccacggcctgccagacttccgaaaggtaataaccatcacagtgcagctctttagttagtccttatcatgtcataaactgtggaccctcgagaatagattacatcactcagataaaagatgtgcgcattatgactcacgtacatgagtccagaacttgtatctacttgtaacgacgtcaagaggattctggaaatggtgcctgctgggctagggacaacctcactagattgctttgctgtttctgaaaggctaatgatgtgatttgtggaaacacgcaggcgattgctaggttcatggggaaagcgagaggaggaggagctacgttcgacccggagcgcattgtaatgagcggcggagccaccggagctcaggaaaccatcgcattttgtctagcgaatcctggggaggccttcctgattccaacgccatattatccagggtacgtagacctatcctacatcaagattttatgttttatgtatatttcacagtgacactaatctgttttaaagaaaactgtttgaggatgagccgatcgaactacggaggcaacattaatataatccagcttactggtataaccaaaaaattagtagtcaatatttgccatcgcacgactgtgacgtcgacaagacagtctcagtatattatatttcttaattaataacgctacaccaaaaccataaccgacctaccggccgcttgaggtttctgcactctccggcctcattatggatctatcggttgatatatatatatatatatatgacagcgatttcacatttcctgcagcttcgatcgagactttcggtggagaactggagttcaactcctccctattcagtgccacagcttcgacaacttcaagatcaccgaacccgcgctagttactgcctatcaaagggcacaaacagctaacatcagggttaaaggaatcctggtaaccaacccttcaaaccctctgggtacaaccttggacagagagacactgagaaccttagtgagcttcgccaacgagaaacggatccacttggtgtgcgacgagatattctcgggcaccgtcttcgacaagcctacctacgtcagcgtctccgagatcgtggaagaggaaccatactacgacagggacctaattcacatcgtctacagtctgtccaaggatctcggcgtccctggattccgcgtgggtgtcatttactcgtacaatgatgcagtggtcagctgtgctcggaagatgtccagctttggactggtctcgactcaaacgcagcacctactggcttccatgctgggagatgatgacttcacaaccaaatttttggcggagagcaggaggagattgtcgcgcaggcacaaatattttactgctggcctccacagagttgatatcaaatgtttggagagcaatgcggggctattctgctggatgaacttgacgcatctgctaaacgaagccacggtggaggcggaactcaagctgtggcgagtgataattaaggaggtgaagctcaacatttcaccggggtcttcgttccactgctctgagccggggtggttcagggtgtgcttcgccaacatggacgataacaccatggaaaccgcattgaagaggatcaggaagtttgtgtcccccgggaatcacactgcggctgcgcaagccaagaagaagaacaagaggtgggacgcggcgctccgcctaagtttgcctcgtcggttcgaggaactgagcatcatgacacctcgcctcatgtctcctcactcgccccttgttcaggccgccaactgatggtgatggatgagcgtgggcgatattaaccgacg

SEQ ID NO: 14 - DNA, 1746 bp, Musa acuminata
  source 1..1746: mol_type = genomic DNA
cttgtctcctgttgcttgaaacttccatggctaagaaaggtgtgccactgtctgagatggcaacttccgacacccatggagaagactctccttactttgttggctggaaggtatacgatgaaaacccttatgatgccgcaagcaacccctcaggagtcattcagatgggattggcagagaaccaagtaagtcctgcatcctaatatcatgacaagtatcttcatttctctggtctaacaattgtcttttagccttcctcaggtttcatttgatctactagaagattatttggagcagcatccacaagaatttggctggggatgtggagtgtcgagcttcagagagaatgctttgtttcaagattaccatgggctcaaaacttttacaagggtaatagctcctgattagtagcagctacatcctgttcgtatatataactcatctaatcttctgcctgcaggcagtggcactttttatggagcaaataagaggaggaaggacacaatttgatcctcaacacatcgttctcactgcgggagctaccgcggctaatgagctgttgaccttcatcttagcagaccccggagatggtctactgattcctacaccttattatccggggtaagagctacggcaaatctgtagatttagagtgtcacttcaccgttctaattggattaacatgacaaagccgcttcttgtgctgtaggtttgatagagatctaaggtggagaacaggtgtcaacatcattccagtccactgcaacagctcaaatggattccagattactctccgggccttggaagatgcgtgtgccggagcagaatccatgaaggttagagtcaaaggactcctcctcacaaacccatccaacccgttggggactacaatcaccagacctgttcttgaagagatactggacttcgtggcgcacaaggacatccacctgatatcagacgagatctactcaggctcagtgttctcctccgacgagttcgtaagcatgacggagatcgtcgaatctcgcggccatcaggaacgcgagagagttcatatcgtgtacagcctctccaaggatcttgggctacctggatacagagtgggcacgatctactcgtacaacaacgaggtggtgacgactgcgaggaggatgtccagcttcacactcgtgtcatcccagacgcagaagatgttggcgtcactgctgtcggacaaggagttcacggagaactacctcaggacaaatcgagagaggcttaagaagaggtacgagttcgtggtggaagggctaagcaatgctgggatcaggtgcttgcaagggaacgctggtctgttctgctggatgaatctgggagagttactcgaagagcccacagtagaaggagagctgagtctttggaacttgatgttgcatgaagcaaagcttaatatatccccaggctcgtcatgccactgtttagaagcaggctggtttagggtgtgcttcgcaaatatgagccagcagacgctggaagttgcactgatgaggatgaaggatttcacggagaagatgaaggctaagcaaatgatttcttcgttgtaaattccctcatgattagagtcatgcatttgtgtcggatgattatatagcaaattcatatacacatgttcaccgtgagactgcctcctctgttctctctcgcctttttccttgttgctgttctttctaaaaccacagaaatggagttcagattcacagaactgca

SEQ ID NO: 15 - DNA, 5331 bp, Musa acuminata
  source 1..5331: mol_type = genomic DNA
atggaagtggcacaggaatggcccgagcccattgtccgggtgcagagcttggctgatgccgaagccatccccgagaggtacatcaagccaccgtccgagcgtcccaatctgaatcccggcacggccatggcggcaggtgagacagaatgccttcccgtcgtagacctcggcgggcttagaggtggcgcggcggagaggcaagcgacgatgcgcgctgtgtcggatgcgtgcagggagtggggtttcttccaggcggtgaaccacggggtgagcccagcgctgacggcggcggtcatggaggcgtggaggcagttcttccatcttcccatggcggagaagcaggcgtatgccaattcccccacctcgttcgagggctacggcagccgcctcggggtcaagaagggcgccattcttgactggggcgactacttcttccttcagctgttaccgcagtccatcaagaactacgacaaatggccaacacttcctgcttccttgaggtacccacacacacactctttctctttcctcatccccgagaggtcacggagcgatgccatcggagcagggagacgactgaggcctacggcgacgaactggtgaagctgtgcggggtgataaaggaggtgctgtcgttaaccctaggaatggacgaagggttccttcacagaggattcggggagcctggcgcttgcctgagggtgaacttctatcccaagtgcccgcagccggagctcaccctcggcctctctccccactccgaccccggtgggatgaccgtgctgctcaccgacgagcacgtcaaggggctgcaggtgcgcaagggcgacgactggatcacggtgcagccgatccctgatgctctcatcgtcaacatcggcgaccaaatccaggttcgcttacttcctcctcctctccctgcatgaggtcacgtaagcgagatagctctgctctctgcatgggatacgcgactaaattacgtacatatccctttacgattagcttatcttctgattattatgccccctttaggtatattttttgcatatttttttatgaatataatatatatgaaattttagaaaggacaaatatgtcatttcagataattttttttgcttcgcgtgcatgcctacgttgcaaatgttactaagccgtaggagaaagatagtgtcaatatcgatcattaaggatatcttatgatgaacataatattgtaattttcttatgatctactaatgatttagcatttagaaattatgaaatatttatattttggattagctgccaataacgagtaagattaaatgcctctaagtagatattataatgattaaagcgtcatatgcaaccaaaagaattaggatgatgagttgataatattagattcttttatttgaacgtcgactatttcttctataaaaaagagaaaaagaaaatgtgacctactacttgaagtggctaatcaatcaactttctctaatttgcacaatccatctaagatcaataaacttcgaattctataagagcatcccgaaagcaaatgatccatcaattaatgtcgtgatacaatgtttaagttgttgatcattatcaatctgttcgaaagcttaggcatgtagatgatacaaaacattttattatgtatataaagaatgaagtttgaggatgaaatgacgaatggttttacctttttttctcatgtgatttgcataggtaaagttgttctttcttaaggaaaaaagtatgtatgcatttccacggtctcattgctacaaaaaactaggtcaactttaagagatagatagcatcatctttccactaattcaacagttcctcctttggtcttatggtgactcaaaagtaccaacaaaaaggggaagaaatgtgcctaatgcaccgaaaagttggtcacgataagatcggcgtagattacaatcaatataataaacgaacagtctaatcatattaaaacatatgcttcgcgtggttgtaagaataattgagtaagcttccaagatcatagtagatatatattatcacttcaatatttcggattatagttcaagtttaacaaattaatgagtcatttatttcatcggatcccatgtcaaaataatctcgaatttctacgtatgtccatggattgaaaagaaggtttccacatatctatctcttttaaatagtatatttacatatattctttaaaatataaatattattggcatacatcccttcatatattagtgttgtgggaaataactttgagccgtggccacagggccgacacggctcggttcgagttcggacgacggggatctccctggggcattcctcgagcccgctgaggcgatcgggtccggtgtccgatcgggacggtgtaaccgtctcctccaggcaggaactcctcgcctgcgcgtccggaggggaccttcggcttcgcacctgcacaaaggtctggccgaggcgctcggcccgactcctccgacgatcaagttagcaaatgtggagggggtttcagatgaagaagtgtttttgtgtgtctgtcccgccccccccccccctcctttctaatgaacgagagagtatttataaggaagcataccgcttcttgagctgcccgcttgcagggggcaggctggtagcgtctgactttgtgttatcgtggcgtgaagaattgagccttggcaagatgttaatgtgcctcgatcggcgttccgatctacattggccaggtgctgttgcgtgaggcatcatctgacgtcagccgagtcttatcataattactatcctcatcatattcccccccgaaggaagtcatgccataaaaagggggggtccgaggcatggcttcggctttgagaaactgtcccagcagggcgccttgccggaggtgtgggaatcgtggagtttagcaactaagaagggtcggatgtgcagtggtgacccaggtagcgtgcggccgacgagcacacttagtagggcaagccgacgcatggtgtgacctcggggagcatggagccgaggaggacgacgtaggcgggctggtcgcgcaggtgtggtctcagggagcatggggccgaggagccgatgagcacgacgcaggcgggctggccgcgcaggtgtgtctcaggagcatggggccgaggagctgagaagcacgacgcaagcgggttggtcgcgtgggtgtgtctcgggaagcatggggtcgaggagccgaggagcacgacgcaggcgggctggccacgcaggtgtggtctcgggagcatggggccgaggagccaaggagcacgacacaagcgggttggccgcgcaggtgtgtctcgggagcatggggccgaggggccgaggagctgagaagcacgacgcaggcgggttggccgcgcgggtgtgtctcgggaagcatggggccaaggagccaaggagccgaggagcacgacgcaggcgggctagccacgcaggtgtggtctcgggcaacatgcaaccgaggagcacgacgcaggcgagcaggccgtcctgaggcagaactcgggctgtctacgaccgaggaacatggctcaagcgggcagtcacccgacattccgggccctccttctagcgccaatctattgtgggaaacaactttgggtcgtggcctcagggtcgacgcagctcggttcgggtccggacgacggggatctccttggggcgttcatcgagcccgctgaggcggtcgggtgcggtgtccgatcgagacggtgtagccgtctcctccgggcaggaactcctcgcctgcgcatctggaggggaccttcggcttcgctcctgcacaaaggtcgggccgagcgccccgacccctccgacaatcaagttagcagatatggagggggtttcaaatgaagaagtgtttttgtgtgtctgtccccccccccgcccccgccccccttcttatgaacgagagggtatttatagggatgcatactgcttcctgagctgcccgcttgcaaggggcaggctggtagcgtttgactttgtgttggcatagcgtgaagaattgagctttggcaggatgttaatatgcctcggtcggcgttccggtctgcattggccaggtgctgttgcgtgaggcgtcatctgacgtcagccgagtcttatcataattactatcctcatcaattagtatcataattcgcccgataataatacttcttgttagcattcatcataaataaaaataaaaaaaattaagtttttttatagaaaaattatgatgaaaagtcaagttgggtatacaatttggattatatagttgcaaaaaaatcaataatagttaatatgagttagtttgagtttaataaattagatgaaattttgagatatcttaatattcttattatctctaatactcttgattagccccatatttttattatttaaaaaaaattattttaactaatgatttaggttgaatgaagttgatagattaattagtttatttgggtcataatatttggtatcattaccgacctaatatttggatatggtgaaaggattcgagtaaaaaaagattatcaataaatggagttagggagattatcgcttgattaatctcatatcttaagtaaataagattaggattaatttataaaaggtttgattggtcataatattatcataactaaattttaaataatataaataccataaggaatttcaattgatactcaaagaaaactaatagatttaatatatatatatatatatgtacataatataatattttgtaataatatatgctacacttaaatttagagaaataagtataaatatgacttgtttatttatttattataaataataattaagtcattactatattcttcaattggagtgaggatgaatatcaaaccatatgatttagtatattttattttattcaaaaatatttatatgaattgtactttatttagtattttatatcgatttaatatattataaaaattattattagaatgatatttaaaatgtcaagataatgatacacgggtaccacagcagagcgtatcacgaatcacgaatcacgaatctcgaagctcgatgatgcaggtgttgacgaatgccacctacaagagcgtcgagcaccgagtgacggtgaacgcgacaacggagcggctctcccttgccttcttctacaaccccgacgacgacctgcccatcgagcccgccgccgagctggtgacgcctacctcgccgccggtgtacaagccgatgacgttcaaggagtacaagatgtacatgaggatgttgggcccctgtggcaagtcgcacgtagatctccacaaggctgcatga

SEQ ID NO: 16 - DNA, 2024 bp, Musa acuminata
  source 1..2024: mol_type = genomic DNA
cgcacatatatgctcatgaaatagcgatgcagagctctctacaagcaaatagacacgcttgctttgtggtcgagcagtgacccaagaatcaaaggattaatccagcaagtataatctccttccatgcaccttgatgacacgtttgtgctcgagttggaggagttgatcgaatatatttgagccgagaacttcgtccatggattgcctgcgagactggccagagccggttgtccgggtgcagtcgttgtccgacagcggcgccaccaccatccctgaccgctacgtaaagccgcagtcggagcgcgcctcggtcgatcccggagacatggtcgggataccggtcgtcgacctcgccatgctaacggacgacgtcgccaactgcgaggccaccgtgacggccatagcggacgcctgccgccagtggggcttcttccaagcggtcaaccacggagtgagcccgggcctgatgaggggcgccagagaggtctggaggggtttctttcatctgcccatggacgagaagcagcgctacgcgaactcgcccaagacttacgagggctacgggagccgcctcgggatcgagaggggcgccattttggactggggcgactacttcttcctccacttcctccccttgtgcctgatggatcacgacaagtggcccgctcttccgcccgccttgaggtaccacatcactgctctgccatcaagctccgatctcctacggctggcttgtcttcgctgccgtcggctggaatccaagcttaacgtgcatgcatgtgcgcacagggagacgagtgacgagtacggcgcggcgttgacgaagctgtgccggaggctactgagagcgctgtcaattggcctgggactggacgccgcctgcttgccggtggcattcgacgacgaaggggtctgcatgagggtcaacttctaccccaggtgcccgcagccggagctcacactcgggctctcggcgcactccgaccccggcggcatgaccgtcctcctcgtcgacgatcacgtcaccggccttcaggtccggaagaacgattcctggatcacggtgcagccagtccccgatgccttcattgtgaacgtcggcgatcagattcaggtgaccgcttcctagtgctcttcctccacttcgtccgtatgcaataaatactgaacgcatcggaaaggcgtggaaataatgttttctttcctccttgttctactgctaattttgtcatcaccggtatcgtcgagcttcctcacatcggagctcaacatgttcttatcctcgttcattaaggcctcgtttcttgtcttatgcgtgaccaagcagacaccacctaataggatctcatgttttatagtgcatttccatttcatcagttgccgtcatggttggaaaaccatcgagtgcttcctgctcaggataagctcggtgatggatggataggcatctctgcatgcggctcagaatggtttgagctgccgcagttactttcctaagactaatggtttttatataagaaggtgggggtgatcctttcaaaggcacgtgttctcgtctgcccccgctgatcttcttctagtccataaacaataagattttggtgtctgttcttcttccacttccacccctgtgagtgacatatctatgcatgcagctgacatctatttgtttgtccagcttaataataatgatacttttgacgggtagaaagatgcatgcgcgctgggtttcattggtggtgatgaatgggttgggttgcaggtgctgagcaacgcggcatacaagagcgtggagcaccgggtgatggtgaatgcggcggcggagcggctctccatggccttcttctacaacccgaagagcgacgtgccgatagggccgatacgggagctcgtcacctgcgatcgccccgcgttgtaccgacccatgaccttcgacgagtaccgcctcttcatccggaagaagggcccccgtggcaagtcgcaggtcgattccctcgtggcagcatgacgacccctctccctct

SEQ ID NO: 17 - DNA, 1711 bp, Musa acuminata
  source 1..1711: mol_type = genomic DNA
ggacggctgtgggagagccgatgggctctatatatggccatgctctgccgaggcagaagcacaacacgagctaattgcagcagggtagcagttggtatacactcttgtgacctctatggctccggtgttgtgctctagcacgagttctgagatgaggatcggagaggtcgaagacatccaggagctgcggcgagctcggccgacggccgtccccgagaggtacgtgcgggacacgaacgagcggccggctctgtcgacgatcctcccctcctctctgagtgtccctgtcatcgacttatcgaagctggtctgcggcaccaaaagacagagccaggaagagatggcaaagctcaccgctgcctgcgaggagtggggcttcttccaggtagcttaatggctcatccaccaacttcttcagcacttattataatggttgggacgctgatcgatgcagcatcaaccatgcgatggcaggtgatcaaccatgggatagagaaagagttgctggagaccatggagagggtggcgaaggagttcttcatgctacctttggaggagaaggagaagtatccaatggcgccaggcacgattcaggggtacggccatgccttcgtcttctcggaggatcagaagctggactggtgcaacatgcttgcacttggtgtggagcctgccttcattagaaagcctcatctctggcctacaaacccagctaatttaaggtacttccatcttgccgtcaccgcaacagagaagaacaagtcttcccctcgcatttccatcagcttctaacatgtatatgcgatcacagctacacattggagaagtactcgaaaagcatacgaaggctctgccagattttgctcatgttcatatcgaggagccttggattgagcccaaactacttcgacgagatgttcggcgtggccgtgcaggccgtaaggatgaactactaccctccatgctcgaggccagacctcgttctggggctcagccctcactccgatggcagcgccctgaccgtgctgcagcaagacacggcatccgtcggcctgcaaattctcaaagacaacgcctgggtgcccgtccaccccatcgccgaagctctcgtcatcaacatcggtgacacgatcgaggtcggcgccatcagccaccctagttttcttctccatcttaatctgccaccaatcctttgctgatcgacgccacatgcacgcaggtcctgacgaatggcaggtacaggagcgtggagcacagagccgtcaccaacaaagagaccgacaggctctcggtggtcaccttctatgctccgagctacgacgtcgagttgggccctgttcctgagctcgtcaatgaccagcagccatgcaggtacaggcgattcaatcatggcgagtacagtcgccactacgtcaccaacaagctgcagggcaagaagaccctggaatttgccaagatacagacaagctactgagcaagaaagccaaactctagacttctccaagtacattcccctactatgtcgacatgtataagcagaatgattagccaagcatgttgtgttaaagatatttacacgaagtgtgtaatgggatgtgtgatcatattaaggtgaatataaagccacccatcttgacttttgaacgcactttcctgtagcttgtcattcgtggtcttgaaaagaaagatgctggcaattatgggtttgaca

SEQ ID NO: 18 - DNA, 1501 bp, Musa acuminata
  source 1..1501: mol_type = genomic DNA
ttacaagagcagcgtagggttactgtctctatggcgacaaccaccacaaggctcctcctcggcgacctggtgtctcacgctaagaacgtcccgcttagatacgtccggccaccctccgcccgcccccacctctccgccgtcgagaagtcgaatgccacgatcccggtcgtagacctgcaggagctctccgggtccggtcgtgccatggtggtcaaggccattgggtcagcttgccaaagcgatgggttcttccaggtaccttcactcgattcgctgcgtgctcttcccaccctctccgtttagtgtaaggggttgatttggatggcaggtcaagaaccacggcattcccgacgacgtgatcggtgccatgttgcgtgtctcgaaggagttcttccggttgccggagtcggagaggctgaagagctactccgacgacccttcgaggacgacgaggctgtcgacgagcttcaacgtgaggaccgaggaggtttgcaactggagggactttctgaggttccattgctatcctctcaaggactacgtgcatgaatggccctccaatccttccgttttccggtagcctccttgcccagcacgtcaagaacaagtactgcgtgcagcttcttaccatgtgccaaatatatctgcagggaggtggtgggtgactactgcaagcacgccaggcaactggctttgaggttgctggaggccatctcggagagcttgggacttgagaaggactacatggagaaggcactggcgaagcaggcacaacacatggccataaactactatccaccatgcccacagccggagctcacgtacgggctgccgagccacaaagaccccaatgccatcaccctactcctccaggacggcgtctccggcttgcaagtcttcaggaacggcaagtgggtggccgtcgaccccatccccaacgccttggtcatcaacatcggcgatcagattcaggtaaaccattcaacaagaagaagaagaagaagaagaagaagaagatgctatactcatatgttcttcctcattccaatcatatctttctttccttcgttcaaaacaggtgctcagcaatgatcgatacaaaagcgtgctccatcgcgcagtcgtcaacgactccagcgagaggatttctattcccaccttctattgcccatctcccgatgcagtaattggaccagctcaagcactggttgacgagcagcatcctgcagtctaccgaagcttcacatatggggagtactatgacgcgttctggaaccgaggcctccaacgcgagagctgcctcgacatgttcagagccaccaacgatccaatctaagccaccctcccaacacaagaaaattccatcagattccaaatcgtgatgacatgatatatacatgtattgtttaatgcgtgtaattgcttgcctttactgtattaatgttaaaccacaaacacataagtcttccattgtgtttgatggctaagacgagcgccaagt

SEQ ID NO: 19 - DNA, 1730 bp, Musa acuminata
  source 1..1730: mol_type = genomic DNA
agcacatacatctcttctgaagcaaactgcccaactggaggtgctcatggattgcctgcaggagtggccggagccgatcgtccccgtgcagtccttatcggaggcgccgacccttcccgaccgctacgtaaagccgccgtcccagcggccctcggtcggcgacgccgcacgcagcctcgacattccggtcgtcgacctcgccatgctgcccggtggcggcgtcgtcgaggcggtgtcggaggcgtgcaggcactgggggttcttccaggtggtgaaccacggcgtgagcatggagctggtgaggaggttccgggaggcgtggaggggattcttccatctgcccatggaggaaaagaagagatacgcgaactcgccgaggacctacgagggctacggcagccggctcggggtcgacgagggcgccaatctggactggggagactactacttccttcacttcctgccttgctatctcaaagaccatgacaagtggcctgcagtcccagcatgcttgaggtaccgcaaaaccctggcttccgctccttcccattagttgattctgactcccgcccacgtgagaccagagaagcgacggacgagtacggcgtggaggtgaggaagctgtgcaggagagtgatgagggcgctgtcgctcggcctgggcctggacgccgaccgcttgcagaaggccttgggcggcgacgacgacggcgtctgcatcagggtcaacttctaccccaggtgcccgcggccggacctcgcgctggggctgtccccgcactccgaccccggcggcatgacggtgctgctagcggacgaccacgtccacgggctccaggtctgcaaggacggtgtgtggatcaccgtccaccccctccccaacgccttcatcatcaacgtgggcgatcagattcaggtaacttcgtcatcgagctctctcctgtcctcatcttgctgtctgttgcgccaaccatggcacaaacctgttttgggcttcctgcgctattactagaggatccatctgaagacaatcatgcacctacaaagtccaaaacataaaccactatcatctgctgcattgtgttcctcgagggaaacacttcgtacaacaagggtcgatgcatttcggttcatcaggtccatgttgagctggccaatgacacccaatcagaccttatggaccactgcacacagtgcaagtccaatcaccgagatatatatatatatatatatatatatatatatatatatatatatatatatatatatatatatgtatgtatatatgtatatatatatgtatgtatatatgtatatatatatatgtatatatgtatatatgtatacatatatttatatatgtaccttattcaatcaaacaatagaaatgcaacattaacacatgtatgtgtgaacgcgtccttaggtgctgagcaacgcagagtacaagagcgtcgagcaccgggcgatcgtccacgccaaggaggagcgcctctccgtggccttcttctacaacccaaggagcgacatccccatcggaccggtgccggagctcctcacggtgaccggccgcgccgccctgtaccggcccatgaccttcgacgactaccgcctgttcatccggcgcaagggccctcgcggcaagtcccaggtcgagtcactcgaggccatggccatcccagggacttgaccggcccccgccccccccgtcgtcgtcctgcttcgcgacac

SEQ ID NO: 20 - DNA, 1384 bp, Musa acuminata
  source 1..1384: mol_type = genomic DNA
ggctatatataagtagcaacgtggagtgacgagtgggaatagacaaaggaaatggcgtgctccttcccggtcctcgacttggagaagctccgtggagaggagagagagcagtccatggacctccttcgtgacgcttgcgagaaatggggcttctttgaggtgctctcattcttttacgtgaacaagttgatgcccacgagcatttgaagctaattatcatggctttccatttgcttgctgatgtagctgctcaaccatgggatctcgcatgagctgatggacgaggtggagaggcggaccaaagcgcactacgagcaatgcaggaagcaaaagttcaaacagttggcgtgcaaggctctcaagagcggacccgggacggatgtcaccgacatggactgggagagcaccttcttcctgcgccatctccccgtctccaacatgtccgacttcccagacatggacgaggagtaccggtaccgcttcgatttccttcgttacagcgcaccccccaccaccatcgactgtagtctgccccgactaaccttcgccttcaggaaggcgatgacggaattcgcgacggggttagagaagctggcggagcgtcttctcgatctgctctgcgagaacctcggcctggaggagggttacctcaagaacgccttctacggatccaaaggtccgaactttggcaccaaggtgagcaactacccgccatgccctcgcccggagctgatccacggcctgcgagcccacaccgacgccggcggcatcatcttgctcttccaagacgaccgcgtcagcggcctccagcttctcaaggatggccagtggatcgacgtgccgcccatgcaccactccatcgtggtcaacctcggagatcagatagaggtcctctctctctctctctctctctctctttctctctctgcgggacaaaagatcaaacaacatgagggcgttcatgcaggtgatcacgaacggcaagtacaagagcgtgctgcaccgggtggtggctcggagcgacggcaacaggatgtcgatcgcctccttctacaacccgagcggcgacgccgtcatctaccccgcgccctccctggtccagaaggaagcggaggcgtacccgaggtttgtgttcgaggactatatgaagctctacgtcacgcaaaagtttcaagcgaagcagcccaggtttgaagcaatgaaggccacggtaacagtcaatggccaacctacgcctacaccttaggacaccacgacgtctcacgtggagatgccaccatctattagaatgtggcatccaattgtggaaataataagcgaagcactatgaacgtggctttttttagtctcgagggttatgtcgtcgatccaattttccacttct

SEQ ID NO: 21 - DNA, 2070 bp, Musa acuminata
  source 1..2070: mol_type = genomic DNA
gcatccattgcagaggaaagttactgagtcttctgtagatcgaggcaggatgattccggtcattgatttctccaagttggatggcgagcagagggctgaagctttggcccagatcgctaatggctgtgaagagtggggattctttcaggtaggctagcggttgcagtctaagaaccgtaaccctgatttcttttatggatgtgttatcgtcaatccttcgtgtctgcagctggcgaaccatgggattgcagaggagctcctcgagcgtgtgaagaaggtctgttccgagtgctacagactgcgagagaaaagcttcagggagtccaaccccgtccggtcgttcaacgagcttgtggatggagaaaccgagggaggggttggtaagcggctgagtgatgtggattgggaggatgtgttcgtcctccaagatggcatgccatggccgtcgaacccaccggagttcaagtaagtagtcgaggaatcgaacagagcaacactgcttcttctctgcgcactgatatatcttggctaacttgcagggagacgatgaaggagttcagggacgagctgaagaagctagcggagaaggtaatggaagtgatggacgagaacctgggcctggagaatggttgcataaggaaagcgttctctgcaaacggcaagcaccagcccttcttcgggacgaaggtgagccactaccctccatgcccacgccctgacctcgtcgacggtctccgggcccacaccgacgccggcggcgtcatcctcctcttccaggacgacgaagtcggcggcctccagatcctcaaagacggccagtggatcgacgtccagcccgtgaagaactccatcgtgatcaacaccggggaccagatcgaggtgctgagcaacggccggtacaagagcgtgtggcaccgcgtgctcgccacccccgacggcaaccgccgctccatcgcctccttctacaacccctccctcaaggctaccattgctccggcgacgaagctcctctcagccgagtccgacagggttcctgcgtcctaccccaagttcgtcttcggcgactacatggacgtgtacgtgaagcagaagttcctccccaagcagccaaggtttgaggcagtggcggcagccatgtgaaactgcagtgcgaccatataagctcagcatcgtatctgcacgtacttgtagggctgttatgagcaatccaaggaggatggaagctgctaagtagtatggtgtgtagatgtgtgtttgcttgcaagagatgcttgcttgaacgcagtggtagatcgcgttctttgttgtcgagtctgtgagtcgctctgtacatcgagcaacttcgactctgtttcttctcctgttgatgatggtgctcttttgagtcgttgatttcgagcttagaacccgtgaattcaagtcgatctccagctttaagttcttaatctactgccaaaatcaatgcaggttggatttggaatcctggaaaccttatgcatggttcgtcttcgaagccggtcaacccttagtctcgctggcaatatccacctttttaatgcaattaatgttcttcttacaagtcaaacagcgctaatgtgagaaaggttgaccggcaagatttggttcgttcctctttgcttcctctgattggtacgtgagagtcaattctcttcatctacaagttgagagcagagggcttcaagcgatccaaacctgtgcagatgctgaacaaactggcggaggaagaagaagaagaaggcgatgctaagcgcttggatgacgtggactgggaggatgtcttcgtcctccaggatagcaaccattggccgtctaatcctccagtgttcgagtgacctaccaattagctgctaattaaagtcgtgtcctctctgtttctgccaatggatcgacgacgatttgctccctacaataacttgcagggagaccatgagggagagaagggaagagctgcggaagccggccgagaaggtgatggaagcaatggccgagaacctgggcttcgacaagagcaataaacccatcttgttcattagtggactttttagggtc

SEQ ID NO: 22 - DNA, 1485 bp, Musa acuminata
  source 1..1485: mol_type = genomic DNA
atggatgacctccgacagtggcctgagccggtcgtccccgtccagtccttgtcggacggcggcctgacctctatccccgagaagtacgtgaaaccgccatccgatcggccctctctcgaggccaatcttgaccgggggctcaccatgccggtcgtcgatctgcgtggcatctacgacgggtcggtggatagccgagccgccatggtggcgatctgggacgcatgcaaggagtggggcttcttccaggtgatcaaccacggcgtgaggccggatctggtggaagagatgaagggtgtgtggagggagttcttccgccgtcccttggatgagaagcagaggtatgccaactccccggcgacctacgaggggtacggcagccgcgtcggcgtcgagaagggcgctgttttagattggggagattactatttccttcatctccttcccctgtccatcaagagccatgaccgacactggccggctcgtccgagcaccctgaggtgtgtagctaccaccgcattagcttgagatttagcttcttgtctgatgattgcgtgggagcaggaaggtcaccgaggagtacggcggcgaggtgttcaagctttgcggggtgctgctgagggtgctgtcgatgggcttaggtttggacgaggagtacttccggagggcgttcggcggcgacggcaccgcctcatgcgtgagagtgaacctatatcccaaatgcccgcagccggagctcaccctcggcctctccccgcactccgatcccggaggcctgacggtgctcctcgccgacgaccacgtcgaggggctccaagttcgcaaggacggcgcgtggctcaccgtccggcctgtccccggcgccttcatcgtcaacgtcgccgaccagatcgaggtcatctgcttccaatcccccactacgatttgcatgcatgacgtacgtgagcacgaagcaagaaagcacgaaaactttgggcacgaaagttggaactgatagctccgatgcttcattggttccttcgaaatgtggccgacacactgtttgcaatactcaacgaagttgacttgcatcaactcctctctttcctaacattacaccatacttgaatcatatcatacatccccctcgccatgccatctgaagacgatgatcgacttcagtcatactccaggatttgagatcatcgtgttcgttttgctcaacaggtgataagcaatgggatctacaagagtgtggaccatcgggtgatagctaactcaaaagacgagcgactctccattgctttcttctacaatccagagggagatgtggccatcggacctgcgccagagcttctcacgccgcagctgcctccactgtatccatgcatcaccttcaacgagtacaggatgtatgtgaggaagagaggcctgagtggcaaatcccaaatgaagtccctcaagctttactgatgtgaagatatcgtaataatgttatcgaatattaag

SEQ ID NO: 23 - DNA, 1374 bp, Musa acuminata
  source 1..1374: mol_type = genomic DNA
tccattgcagaagggtgtttcccagtcttctgtagctttgaggcatcatgattccagtcattgatttctcgaaggtggatggcgaggagagggctgaaaccctggcccagattgctaatggatgtgaagagtggggcttctttcaggttcgttagcttgcagttggtgagtgtaatggtttcttctcttggacgtcttctaaccagtgttttgcatctgcagctggcgaaccatggcattccagtggagcttcttgaacgtgtgaagaaggtctgttctgcgtgctacaagttgcgacaggagagcttcaaggaatcaaaccccgtgcagttgctgaacaagttggtcgaggaagaaagtgagggaaggaatgtggagcggctgaacgacgtcgattgggaggatgtgttcgtcctccaagatgataagccctggccatctaatccccctgagttcaagtaagaacacaaggacgaggaatcaaaggagagaagttcaatggatcgagtcactgatgcttcttggctaacttttcagggagacgatgagggagtacaggaaagagctgaggaagttagccgagagagtaatggaagccatggacgagaacctgggactggagaggggctacataagcagagcattctccgcaaacggcgagcacgagcccttcttcgggaccaaagtgagtcactaccctccctgcccgcggctcgacctcgtcgacggcctccgcgcccacaccgacgccggcggagtcatcctcctcttccaggacgacgaggtcggcggcctccagatcctgaaggacgacaagtgggtcgacgtgcagccggtgaagcactccatcgtgatcaacaccggggatcagatcgaggtgctcagcaacgggcggtacaagagcgtgtggcaccgcgtgctcgtctcctcccacggcaaccgccgctccatcgcctccttctacaacccttccctcaaggccaccattgctcccgccaccaagcttgtcgcaagccagccccgggaggttggtgcttcgtatcccgagttcgtgttcggggactacatggacgtgtatatgaagcagaagttcctccccaaggagccaaggtttcaggcggtggcagcagctctgtgaaaatgcaggaaggagatgatacactccagggtagtttaatgtgtgaccatctaagtttatcagtgtcgtatatttataggtcggtatcagcgacagatgcttgcttgcttggacatgtgcagcacatctgtatgatacaagtactgcgtactgagtctgttgtcgagtctgtgtgctttgcttcgtacagtacctggagcctatattccaagttgtgtcaggtattataagctctt

SEQ ID NO: 24 - DNA, 1259 bp, Musa acuminata
  source 1..1259: mol_type = genomic DNA
gtagctgcacatcgagtcaaggagaggagcaaagccatggaggtccctgtgatcgaccttgcggagttcgagagtgaggagaggagcaaagccatgtctcgatttcaccaagtgtgcgggaattggggcttcttctgggtaatatgatctctctgcttcttgctcttgattcgattcggtaagtcattcgatactggcttcttcaacgcaggtcgagaaccatggagtagctgtggctttgatggaggagatgaagagacatgtgtactcccactacgacaagtgcctcaaggaaaggttctacgactcggagttggcgaagggactcgggcctcaaaccgatgccgcagaagtcgactgggagaccacctacttcgtgcagcatcagccggaatcaagcacggaagacgacctcggcctcggggtagaattccggtcagtctccagcctcagactagtttaacggcaggaacaagcgcttacaggttcattcgatcgatgtcgcagcgaagccatggatgcttatgtcagccaactgaccaagctcgcggagaagctggcggagttggtcagcgagaacctgggactggacgatgatcatctgaagaagacatttgcgcctccatttgtgggcacgaaggtggccatgtacccacagtgtcctcagccggagctggtgacgggcctccgcggccacagcgacgccggcggcatcatcctgctgctacaggacgacacagtcccaggcctggagttctacaaggacggggaatgggtgccggtgactccgaacaaaggaaaccgcatcttcgtcaacttcggcgatcaggtggaggtggtcagcaatggcttgtacaggagcatgtggcaccgggtgctggccgataagcacggcagccggctctccgtggcgacgttctacaatccgggcggcgatgccatcgtcgggccggctccgaagctgctgtaccccggcggataccggttccaggactacctccattactacttcgggaccaagttctcagacaaaggagcaaggtttcaggccgtcaaggaaatgctcgagtgaaggcctcgtggcttaagcaataagagtgttctcccgcatttaagactaccctgttctgttctgttccgttccgttccgttctactgtgtctttgacatcaacaaaattggtatgatttagatctgagaaggttatgagctatgcttgaatcaatgcagaatgaatgaatggtatgcgctgttcgaac

SEQ ID NO: 25 - DNA, 1691 bp, Musa acuminata
  source 1..1691: mol_type = genomic DNA
tgcggttgtcgtccccaagattgcttcgacgccttggagttgtagtctcatggattgcccgaaaggatggcccgaacaggtagttcgtgtccaggccttgtccgacagcggtctgatgacgattccagacctgtacgtcaagccgccggccgagcgcccgtcggttggtaacggtggcgacgttacgtccgacatcccggtcatcgaactgggggggctggcggagggcgcggcggagtgccgcgccaccatccgcgccgtgggggacgcgtgcagcgagtggggattcttccaggtggtgaaccatggggtaagcccggacctcgtcgccagggtccgggaggtgtggcgggccttcttccatctccctatggaggagaagcaagcttacgctaatgaccccaagacttacgagggctacggcagccgcgtcggcgtcgaaaagggtgccatattggactggggtgactacttcttcctccacctcctccccgaatccatcaagaaccagaacaagtggcctgccctgccatcgtcttgcaggtacagtacactccattgtcatataacagtactagtaacgacggaaaaccatagtattcatggacatgcatgcgcgtgatcgagcagggagacggtgcaagagtatgcagatgagttagcgaagctgtgtgggacgctgatgaaggcgctgtccataagcttaggcctggacgtggagcagctgcagaccgccttcggaggggacgccgtcggcgcctgcctccgcgtgaactactacccaaggtgcccgcagccggagctcaccctcggcctctccgcccactccgatcccggtggcctcaccatcctcctcgccgacgactgcgtcaacggtctccaagtccgcagaggcgacgactgggtcaccgtccaacccatccccggcgctttcatcgtcaacgtcggcgaccagattcaggtatagccccgatccaccttgtggcggtacgtgtgtcgtgcatctcttagcgactactttgttcggtgatggttatgacgtatcttatttacgtatggccattcggatgcacgagtccgacatcccccatccctctgtggatgacgcgaggttttgtcttcatataccgtgtgctttgtcctacctagttttggacacttgccgccatcgctgttcgccctctggcgctggtgatcgatggctatcttaatatttggtcaacatccgaaacacatgggccgggttgaccgcatcacagtgacttacaaaacaagtctacctaagccgcccacgtcggatgcgatgcacacgatggatgtggaaacggcagcagcaggtttaacctgcgtttcatttggttgcaggttctgagtaacgcagtgtacaggagcgtggaacaccgagtggtggtgaacgcagcacaggagcggctctcgctggccttcttctacaatccgaggagcgacgtagcgatcgcgccggtgagcaagctggtgacgccggagcggccgcagctgtaccggccgatgaccttcgacgagtatcgtctgtacattaggaagaaggggccgaaggggaagtcgcaggtggagtcattgaaggcacagagtgttaattgatcaggtgtacgtcatctgcttgctgtgatatgtccacatgtagcgagccatggttgcagatcttgcttggg

SEQ ID NO: 26 - DNA, 1520 bp, Musa acuminata
  source 1..1520: mol_type = genomic DNA
atggactgccttcaggaatggccagaaccggttgttcatgtccaggccttgtcggacagcgctctgacgacgattccagacctgtacattaagccgccgtccgagcgcccgtcgtcggacaaaggcgtcgccacgccccacatcccggtgatcgacctgggagggctggcggagggcgcggctgaatgccgcgccaccatctgcgccgtggcggacgcgtgccgctcctggggattcttccaggtggtgaaccacggggtgagcccggacctggtcaggaaggtccgggaggtatggcgaggcttcttccgcctccccatggcggagaagcaagcgtacgccaacaaccccaggacttacgaaggctacggcagccgcgtcggcgtcgaaaaaggtgccatcttggattggggtgactacttctacctccacctcctccccgagtccattaagaaccaagacaaatggcctgccctgccgtcttcttgcaggtgcatatcaagcgcaataactcatatgacaggacagtaagaacggaataagcccaattatatggacctatatttacaatggacgtgcatgattgtgatggaacaggcagacggtgcaggagtacggagacgagatggtgaagctgtgtgggacgctgatgaaggtgctatccataagcctgggcttggacgtggatcaactgcaggccgccttcggaggcgacgacgtaggcgcctgcctccgcgtgaactactatccgaggtgcccgcagccggagctcaccctcggcctctccccgcactccgacccgggcggcctcaccgccctcctggctgacgactgcgtcaagggcctccaagttcggagaggcgacgattgggtgaccgtccagcccgtcgccggcgctttcatcgtcaacatcggcgaccagattcaggtgctctcgctctctctctctctctcggcgattcctcgaggtcaaagttttagctgttttgttcccgcggatcttttcgtcgtccagggaaactggagtcgcatgcaagcatatctcaaccatgtcctgtgagacgacgcttgtctgcaaagttgtcttccctccgaaaccttcctcggtcactctgacaaccttcctcttgcggtgtttgttgtcagctttactttatgattccgttgacccatctcaccacccagcttgtgtcttctgccacttgttccaatcatacgtgggtaaatatatatatgtatatatatatcttatatttcttgtgttaatgctacagattttgagtaacgcaaagtataagagcgtggaacatcgagtgacagtgaatgcagcgcaggagagactgtcgctcgccttcttctacaatccgcggagcgactggccgatcgcgccggtcggccagctcgtgacgccgcagaggccgccgctctaccaggcgacgaccttcgacgagtaccgcatgcacgtcaggaagaatgggccgacggggaagacgcaggtggaatcattgaaggccatatga

SEQ ID NO: 27 - DNA, 1402 bp, Musa acuminata
  source 1..1402: mol_type = genomic DNA
acactccagatagaaagcacaagtgcaatcagggaagaaagagcgtgtcatggattcctttccggttatcgacatggagaagcttttgggaagggagagaggagaagccatggagatcctccgagatgcttgcgagaaatggggcttctttgaggtgctgaagcatacataactggttttgcttctttgaactatatatatattgctaaaatgtactatttgcacatgcaatctgtgtgtagattttaaaccatggcatctcacatgacctcatggatgaagtggagaaggtgaacaaagaccagtacaacaaatgcagggagcaaaagttcaacgagttcgccaacaaagcactggaaaacgccgactcagaaatcgaccacctcgactgggaaagcacctttttcctgcgtcatctccccgtctccaacatttctgagatccccgatcttgatgaccagtataggttgcacgatctgatcatgatgtcatcttctggcctggtcttttcaccttgctcatcgtttcgtttcttgggacgatgactgcgtgcaggaaggcgatgaaggaatttgcggcagagatggagaagctggcagagcggctgctcgacttgctgggtgagaacctggggctggagaaggggtacctgaagaaagccttctctaatggatccaaggggccaacctttgggaccaaggtcagcagctacccgccatgcccgcgcccggacctggtgaagggcctgagggcgcacaccgacgccggaggcatcatcttgctcttccaggacgaccaggtcagcggcctgcagttcctcaaggacggcgagtggctggacgtgccccccatgcgccacgccatcgtcgtcaacctcggcgaccagctcgaggtttgggtcctctttgctctcgtttccgctgcccgtcgtctgtgatgttgaatgcaacgaggtctgcaggtaatcaccaatggcaagtacaagagcgtggtgcaccgcgtggtggctcagactgatggcaacaggatgtcgattgcctccttctacaaccccgggagcgacgctgtgatcttcccggcccccgctcttgtggagaaggaagcggaggagaagaaggaggtctatccgaagttcgtgttcgaggattacatgaagctctacgtcgggcataagttccaggccaaggagccaagattcgaagccatgaaagccatggaagcagttgccacccacccaatcgctacctcttaagtgacagcccccaagttagtgcatgtcgctgtacttcgcgttaggaagctgtcgtctatgtctatgtaacccgatggatgtgtggtatgtacgtgtgtgagccttttctaatgaagcaaatcatataatatatatatatatatatatata

SEQ ID NO: 28 - DNA, 1225 bp, Musa acuminata
  source 1..1225: mol_type = genomic DNA
gctggtgaatgcatctactacggatgtgaagagttgggtcgaggaagcgtgcttaccgagtcggaggaataacccgagaggcacgaaagccggcggaaatggagatcccggtgatcaaccttggagagctggagggagagaagagaagcaaaaccatgtcgctcctccatgatgcgtgccagaagtgggggttcttctgggtacgttgtgagcatctttatctctgcaagcattggtattcgtgtttggttactctgatgagtccggcatggcagctcgagaaccatgggattgaggatggagtgatggaggaggtgaagcagctggtgaagcagcactacgaggagagcatgagggagagcttctacgagtcggagctggcacagggactgcgacgtggaactaaagcctcggatgtggactgggagaccagcttcttctaccgccatcgcccggatcccaacatcaatgatctccccgaactggttcggtgagttctcttccatggagtataaccacgtagagcaaccccaagctgacgccgcagcatgctcgtgcagtgacgctatgaagcaatacgtcgaacaggtggtgaagctggccgagaagctcgcggagcttctgagcgagaatctcgggctggcgaatacctacctgaagaacgcattcgccgagcctttcgtggggacgaaggtggcaatgtaccccaaatgctccaacccggagctcgtcatggggctccgcggccacaccgacgccggtgggatcatcctgctgctgcaggacgacacggtccccggcctggagttcctcaaggacggcgagtgggtggcggtgccgccggcgcagggtcaccgcatcttcgtgaacctcggcgatcaggtcgaggtcgtgagcaatggcgtctacaagagcatcaggcaccgggtgctcgctgacgggaccggaagccggctgtcgatcgccacgttctacaacccgggggccgacgccatcatttccccggcggccgagctggtgtacccgagtcgctaccgcttccaagactacctggattactacaccaagaccaagttctcagacaaagcgtcgaggtttcagaacatgaagcagacgctcgtgtgagccactcatgcctgtagtagctgacggaagaggaatttgtactggtcaatccacgcttgtgcttcaatccaaataaacatcgatcgccatctcttcttta

SEQ ID NO: 29 - DNA, 2108 bp, Musa acuminata
  source 1..2108: mol_type = genomic DNA
atgaacgtagtacaggagtggcccgagccagtcgtccgtgtccagaccttggccgatgcccaggtaatccccgagaggtacatcaagctaccatccgagagaccacacccttcttcagcggcaggcggcgcaggaagccttcccatggtcgacctcggcggcctcaagcgtggcgcagcggagaggcaggcgaccttgctcgccgtgtcggatgcatgcagagactgggggttcttccaggtggtgaaccacggggtgagcttggagctgatggccaggatgagggaggtgtggaaggggttcttcgatctccccatggaggagaagcaagcttacgccaattcccccgtcaccttcgagggctacggcagccgactgggcgtcaagaagggcgccattctggactggggagactactacttccttccgctgttccctcactcgatcaagaactacgacaagtggccttcccttcctgcttccttgaggtatatatccacgtagattcacagagatccatgcatgcatgttcctctacacttttctggtcttcatcatcatctgatgatcagggaaacgactgaagaatacggtgaggaactggtgaagctgtgcggggtgatacagaatgtgctctcgttaaccctaggattggacgaagggttccttcacagggaattcggagaagctggagcaggactgagggttaactactatcccaagtgtccgcagccggacctcaccctcggcctctccccccactccgacccaggaggtttgaccattctcctcaccgatgaccaggtgaaaggtttgcaggtgcgcaagggcggctcatggatcacggtggagccgattcccgatgctttcgtcgtcaatgtcggcgaccaaatccaggtttgcttcctcctatatggttcatgtttttgccttgatcctttctcatctgcatgcacgtcgatgtgtgtgtgatatatgaggaagtgttcttagagattcgatcgaaacagtgctctttcgcgttgcagtgtccatccactgcatgcagaagctgtgcatgcatggacatgatagaattcatgctctaagctgtgcttccaaaatatgccaaaactgagacaacaaaaaaggttgtgcaaaatactcgaaatttcgatactaaatgcaataatttttctcttctaattaatacactaaatttaatcataatataatgccatatattaatacacaaaaaaaaccacgaagaactctgaaatatctaagatagtcaaatgtttcatatgcgcgggagaagcttaattataataccagtgtctaagtgtttggtcacttcatccaaataatattaacatgcatgtcaaaaatcttctaaaagaatcatcaactaagaacagggggtagatagataagatttggatgataactaaacatcgggaaagaaacttgtgatttgcatcgataaggctatcttctaccttttgtaaggtaagtgtccagagcatgcagccacgtgctcatctctccttcttcacgcccttctttccatctctagcatgttcttccttggtgatttgactgttaacctaaagtcctgtcaacgcttgatagatttgtgccatcatctctctctctctctctctctctccctctcgttatctttccaatcacagaaacgaaaccatatgctttttaatgcacctcaaaagttgctctcattgagttcatgtgttctagctgtgtgtgagatggagaggaagagagagaggctttgattacttgggaattgcatgctcttcttggccacgcaggtgctgaccaatgggaggtacaagagcgtggagcaccgggtggcggtgaatgcagcaacggagaggctctccatggctttcttctacaacccccaagatgacttgctcatccaccctgccaaagagcttgtggcagatggcacatcccccatgtacaagccgaagaccttcaaggagtacaagctgtgcatgaggatgttgggcccttgtgggaagatgctggccgacgccatggaagctacttaattaataagcatcagaattgagggataccaaacaattcgttcagcttcaagg

SEQ ID NO: 30 - DNA, 1338 bp, Musa acuminata
  source 1..1338: mol_type = genomic DNA
atcgatcaccattcgagaagcagtatagtagcacagttggtaaccggatcaccccatctgtcttttggagaaatggccgttccaatcatcgatttctcgaagctggagggggaggaacgagccgaaacattggcacagattgccactggatgcgaagaatggggattctttcaggtctgttatcatggctttgttttctttttccgcgggtcctcttctttctccttccgatgttcttatgaagtcgatgcgtttgcagctggtgaaccatgggattccggtggagctcttggaacgcgtgaagaaggtgtgctcggagtgctacaggctcagagccgagggcttcaaggggtcgaagcctgtgcagctgttgaacaagctggtggaagaagaagaagacgaagctgccgacgctaagcgcttggacgacgtggactgggaggatgtcttcctactccaggatgacaatgagtggccgtccaacccaccagagttcaggtaatcatcagcttcctatcgggacttgttaggctgattgatatgtggctgtactccgtctgtcctagtgctgaaagtttgcacgatcatgcagggagaccatgaaggagtacagggaagagctgaggaagctggcggagaaagtgatggaagtgatggacgagaatctgggctttgagaagggctccatcaagagtgcattctccggaaacggggagcatcatcccttcttcggcaccaaggtgagccactacccgccgtgcccacgcctggacctggtgaacggccttcgcgcccacaccgacgcaggcggcgtcatcctcctcttccaagacgaccaagtgggcggcctgcagatccttaaagacgggcagtggatcgacgtgcagccagtggccaatgccatcgtcatcaacacgggagaccaggtcgaagtcctcagcaacgggcggtacaagagcgtgtggcaccgggtgctgacgaccagcgacggcaaccgtcgctccatcgcttccttctacaacccctccttgaaggccaccatcgctccagggaccaacgaggacgactctgctgcagcactgtaccccaagtatgttttcggggactacatggatgtgtacgtgaagcacaagttctcgccaaaggaaccccgctttgaggcagtcaaagctctgtgaggatcgaaaaatgcataattgttggaatttacttctcatatatatatatatatatgaatgattctttgtggtgttttatgaacatgtgtaatttaattaatggttttgttttgacttggcataaataaaataaaaaaaaatatgttttgatttatacatt

SEQ ID NO: 31 - DNA, 1761 bp, Musa acuminata
  source 1..1761: mol_type = genomic DNA
ccaatttgtcttctcttatagctttatgttcttatttgtatgtagcgttccctgcaaacgaggagaagaacacttactgatcgcaacgcaatggcaacgaaggagaattccggcactgcagtgatcgaaggccgcgtcgaggacgttcaagagctacggcgctctcatccgacggtgatccctgcgcgctacgtgcgagatggcaacgagaggccttctcctgctctctcgcccggcctcccttccatggacgtccccgtgatcgacttatcgaggctgggcagctgcagcagcaaaacaccagagcgtgaatcagagatggcaaagctcgctgctgcctgcgaagggtggggcttcttccaggtgcgtactgcgcttcttcatctctcttctggttccccagaaaccgaagcagcactgaggcgatgacacatgcaggtaatcaaccatggagtggagcatgagctgctagagaagatggagaagctggccaaggagttcttcatgctgcctttggaggagaaagagaagtacccgatgcctcccggtgggattcagggttacggccacgccttcgtcttctcggagcagcagaagctggactggtgcaacatgtttgcgctgggcctcgcgcctgccttcatgagaaagcctgaactatggcccacgaatccaccttccttcaggtaacacatcgccgccgtgtttctctcgccatggctccgattcatacctgtattactgctacagcgagacactggagaagtactccaacagcataagactactatgtgagacactgctcggcttcatcgccgagagcctcggcctccgccgcagcttcttcaacgagatgtttggggaggccgtgcaagctgtgaggatgaactactacccgccatgttcgaggccggacctcgttctggggctgaccccgcactccgacggcagcgccctcaccgtcctgcagcaagagacagcatccgtcggcctgcagatcctcaaagacggcgcctggcttcccgtccatcccatcgccaacgccctcgtggtcaacgtcggcgacacgctagaggtaagagctccgtgggaagccgtatgcgctcaatccagcgcgggcgatcactgacgtgacgagacatgcaggtgctcacgaacggcaagtacaagagcgtggaacaccgagcggtgaccaaccgagagagcgacaggctctccatggtcacattctacgctcccagctacgagatcgagttgggtcccgttcctgaactggtgaatgacaaggcatgcttgtataggagatacaatcatggcgagtacagtcgcctctacatcaccaacaagctggaagggaagaagaggttggaatttgccaagattcagacgagtctctgagcaagaaggtcatcatctccaaattaatcgcattcccctccacaagtctgtatatgcttatgcatgatttgtattagatgagttcttactcgtcgagcatggtgtcacatcgtatacatgcagtgtatatatggggggtgtagaaattggattaatgtgacaccaactgcatcgtaatgtatcaaacacaccaccatcatttccctttctgtagcattccatggttcacatcccacttcaccaaattcatatgttaatatgtagaaagtagggtgactcatctgcatgtatcatccacatccctgacatagctgatcattttacatgctacaagcaaagcaagcatatatactatagagaacc

SEQ ID NO: 32 - DNA, 1296 bp, Musa acuminata
  source 1..1296: mol_type = genomic DNA
ccattcgagaagcaatacagaagcataatttgcaaccagagcaacatctcgtcctcgctagaaatggccattccagtcatcgatttctcgaagttggaggggaaggaaagagctgaaaccttggcacggattgccaatggatgccaagaatggggattctttcaggtttgcatcccatttgtctggttccttctttctccttactgggatcttttcgagttgacgctggtactaaagcagaggaatctacctgacctgtttgcagctggtgaaccatgggattccggtggagttcttggaacgcgtgaagaaggtgtgctccgagtgctacagactcagagcggagggcttcaaggcgtccaaacctgtgcagctgttgaacaagctggtggaagaagaaggcgacgccgccgatgctaagcgcttggataacgtggattgggaggatgtcttccttctccaggatgacaacgagtggccggccaaccctccagagttcaggtgatcatcaacttccacgcagggctcgtcaggctaattgatatgtagttataagtgcctaacgtatgccctcttcatgcgcaatcttgcagggagatcatgaaggagtacagggaagagctgaggaagctggctgagaaggtgatggaagtaatggatgagaatctggggttcgagaagggctccatcaggaactcattctccggaaacggcgagcatcaacccttcttcggcaccaaggtgagccactacccaccgtgcccgcgcctggacatggtgaacggccttcgcgcccacaccgacgcaggcggcgtcatcctcctcttccaagacgaccaagtgggcggcctgcagatccttaaagacgggcagtggatcgacgtgcagccagtggccaatgccatcgtcatcaacacgggagaccagatcgaagtcctcagcaacgggcggtacaagagcgtgtggcaccgggtgctgacgaccagcgacggcaaccgccgctccatcgcttccttctacaacccctccttgaaggccaccatcgctccagggaccaacaaggacggctctgctacagcgctgtaccccaagtacgttttcggggactacatggatgtgtacgtgaagcagaagttcttggccaaggagccgcggttcgcggcggtgagagccgtgtgaggatagcaaaagtgcacgttattcattaagatatattgttccttcgattgaattcttcgcatgagaagaacgtttgtttgcatcagattaattcttcatgtaatgaataaaacgagt

SEQ ID NO: 33 - DNA, 1227 bp, Musa acuminata
  source 1..1227: mol_type = genomic DNA
agcaatacagaagcataatttgcaaccacagcatcatctcctcctcgctagaaatggccattccagtcatcgatttctcgaagttggaggggaaggaaagagctgaaaccttggcacggattgccaatggatgccaagaatggggattctttcaggtttgcatctcatttgtccggttccttctttctccttacagggatcttttcgagttgaggctggtactaaagcagaggaatctacctggcctgttttgcagctggtgaaccatgggattccagtggaactcttggaacgcgtgaagaaggtgtgctccgagtgctacaggctcagagcggagggcttcaaggcgtccaaacctgtgcagctgttgaacaagctggtggaagaagaaggcgacgccgccgatgccgagcgcttggataacgtggattgggaggatgtcttccttctccaggatgacaacgagtggccggccaaccctccagagttcaggtgatcatcaacttccacgcagggctcgtcaggctaattgatatgtagttataagtgcctaatgtatgccctcttcatgcgcaatcttgcagggagaccatgaaggagtacagggaagagctgaggaagctggctgagaaggtgatggaagtaatggatgagaatctggggttcgagaagggctccatcaggaactcattctccggaaacggcgagcatcaacccttcttcggcaccaaggtgagccactacccaccgtgcccgcgcctggaaatggtgaacggccttcgcgcccacaccgatgcaggcggcgtcatcctcctcttccaagacgaccaagtgggcggcctgcagatccttaaagacgggcagtggatcgacgtgcagccagtggccaatgccatcgtcatcaacacgggagaccagatcgaagtcctcagcaacgggcggtacaagagcgtgtggcaccgggtgctgacgaccagcgacggcaaccgccgctccatcgcttccttctacaacccctccttgaaggccaccatcgctccagggaccaacaaggacggctctgctacagcgctgtaccccaagtacgttttcggggactacatggatgtgtacgtgaagcagaagttcttggccaaggagccgcggttcgcggcggtgagagccgtgtgaggatagcaaaagtgcacgttgttcattaagatatattgttccttcgattgaattctt

SEQ ID NO: 34 - DNA, 1561 bp, Musa acuminata
  source 1..1561: mol_type = genomic DNA
atggaggtggctgaggaatggccggaaccaatcgtccgggttcaaactttagctgatgccgaagctgtccctgagaggtacatcaagccaccgtccgagcgacccaacctgaatcccggtacggcgttggcgccgagtgagacgggaagccttcctgtcatcgacctcgccggcctgagtggtggcgccgcggagaggcgggcgacgatgctggccgtctcggatgcttgccgagactggggtttcttccaggtggtgaaccacggggtgagcccggagctgatggaggggatgagggaagtgtggacggcgttcttccggctacccatggcggagaagcaagcttacgccaactcccccaagacattcgaggggtacggcagccgcctcggcgtcaagaagggcgccattcttgactggggcgactacttcttcctccagctttcacctcactcgatcaggaactacgacaagtggcctgttcttcctgcttccctgaggtatacatatacacacatggatccttgtttccgctctttcgatcatttggatgctgcgtactgatattgaggatgcgagcagggcgatgacggaggcctacggcgaggaactggagaagctgtgtggggtgataaagaaggtgttgtctgcaaccctaggactggacgaagagttcctccacagagcctttggagaggctggcgcttgcctgagggtcaactactaccccaaatgcccgcagcctgatctcaccctcggcctctctccccactccgaccccggagggatgacggtcctgctcaccgaccaccacgtcaaaggccttcaggtgcgcaagggtgacgactggatcacggtggagccggtccccggtgctctcatcgtcaacatcggggaccaaatccaggttcgcttcctcccggaccattgcatctatctcacgcatacgatacgtcctccgcctcggcctgcatgagtatagccacgatggacgtgaataggacgcatggtcttaaaaacctatttgttttcttatctcaattgcgtgattggcatgacaacaaagtctcatctttttctgtcctgatgcggcatgattcttcctccctgcatccaaaaataggtcaactttaagatttttggtaagattcttccccgctgcatccaaaaataggtcaactttaagatgtttcgtcaaatcgttgtcttcggaaagcaccaaaaacgtgtcttatacgaacgtagaatgtaaaaggacaagagatagtttactagtgcagttggctgtggtgataattcaacctcgatgacgcaggtgttgaccaatgcgacatataagagcgtagagcaccgggtggtggtcaacgcggcgacggagcggctgtcgatggccttcttcttcaaccccaacgacgacctgccgatccaacccgccgccgagctggtgacgcccgaggcgccgcccctgtacaagcggctgaccttcaaggagtacaagctgttcatgaggatgttgggcccccgtggcaagtcccacgttgacttcgtcaagtccacctga

SEQ ID NO: 35 - DNA, 5306 bp, Musa acuminata
  source 1..5306: mol_type = genomic DNA
cgttcgtccatggaagccgcggccgaaacccaacgcgtccaaaccctcgtggaggccggcgtcgcccacctccctgcccgatacgtccagccgccggagctccgcccgcacctcagccgccgtcgcgatgccacggcggattgcggcggcattcccgtcgtcgacctcggcccctccggcggcgaccccgtcccggcgatcggccgcgcctgccgggagtggggcgctttccaggtggtgaaccatgacgttcgcccggggctcctggaggaggtcagggccatggggtcttccttcttccgcgcccccatggaggccaagctccggttcgcgtgcgatccccggtcgccggcctccgagggttatgggagccgcatgctcgcgaaggacgatggggtgctcgattggagagattacttcgaccatcacgcgctgccggagtctcgccgcaaccctagccagtggccggatttcccatccaattacaggttaggatagttggattgaaattatcaaccttgtgcatcttttttcttttagaattgattcaaacaaagctcgtagaaggttgcaaatgagcaagtaagcatcttttagttaagaagacgtccgagatgggttttgatccgactgggatttagtgatttcgataagggatgaaaggtggcaggtctctggggttttgagttcacctaccagcgctgcatgttgattggtcatactgaaattgaatgtttaattttgtcatttctatagggaaaaactgttcaataagatattcatggtatgcaaccatttgaacttttgcgagaaatggtatttctaaaactacttaatgatcgagtatactatggtagattggatttgcatgtgttaagtatttaactcgttcggacaaagaaatctttcattctgtgcaatctttcgtttaccatctactatattatttggaaggtttagcggaggcgccgctggctaaagtttagttgttatttgttagtttctcaaaaatcagctctttgacttgtttgatatttttattgttgaaattcgcttagtaattgaaggctcggaactaatcagtgaaaaactagaataatttagttgtttgcacagtgatgatatgtctctgttttacttataatgtaatttactgatatatttaataagtttcaatggcctgcatattgttgctgctgatattatcctggtaacatttgaagatcacaatttaaagcaaacttcatttttgggtgaaaagtctttgaagaataagaaccagctaacatcagaaagcaatagagtaaatagatgcatttttagtggagtagtgaaatcttggtcatgcgtaataccactgagacactcagggtgtgtgtcgttcatcttgactgatgaggaagcaattcctttaaattgagttctgttttctttaggctgcagtcagttcgaagaatttagtcaagttctagttagttatagacctcagactttgaactcagagttaagatgtcaaccaactggatatgacacctaaaggtcacaaggatcttgcttttgtgatattgtttttgaacagaaatgagaacctaaaattttgttggtttgagattcaaatttgatgatggagggactcactttgtgtagtgaatctgaatccaaaaaggaaattttctggaacggacaaaataatccattgaagctctctatgacttctcaattagaggaaactttcttaatcttagcttcaggactcttttcaagactggcatggaactactaattaaaatggtcatctcctgtgcatcaaaaatttgagcctctcattctggatcatttacattatacaaaattttagaccttgattggttttctactgcagttctgaatatcattactaaaaaaaaaatgcaatgtgatacgtgtgagtcatattgctaaatgtttccttcagctacataaattcaggcattaatgccaccgttctctttttcatttctgtccagcatgaacttgtgatgccttctaatgcatgcaatagaactggctgatttgggcagggatgttgtgatagaatatagcaacaacatgaagaagcttgctcaaacattgttatgtatgatctcccaaagtcttgggttaccaccactgtacattgaagaagcagttggagaagtttatcagaacataactattagctactaccccccttgtcctcagccagatcttgctcttggtttgcaatcccattctgatatgggtgccataacacttctaatacaagatgatgtggaaggtcttgaggtactgaaagatggggaatgggtgcaagtacagcctttatctgatgcagttgttgtcattttggctgatcaaactgaggtatttgcatttaagttcaattatgatgccaaaatgttatgtatctgtaactgtttttgttgtaagctctccttcaaattaatactgatttatcttaaatgattgttagaacatttagtttattgatattctataatttggtcatttggtagagaattttgaatgtttctagatgaatttattgattctaaatgtaacaataacttcacatgtaactgcgttttgcaaagattcaaaggcatgaacaggtagttatatatcttagatttctaaaggttacagggactgatcatatatttctaggtggtagaccagcatcttaatcgacacttcttaccacattagatatcctcttgctctttgacaaatattaagtattgctgttcttcattaattattttctctcttttttcttgacataaaaattcattttcataaaaacaagtgttataataactaggtaatgcttacttttataatctttgtcttgattaattatactaatttttgctccttgtatgaactaaggatgtacatgttagttgtgattgttccgtttaacacattctaaaatctacatatcacatatgctaacatttccatatatgaacaactgattcatccattgcactatcagttcatgtaaagccactgcatgaacttgatctaatgagctgttggtttgaagtatattaatagttgtaatctctgtaataatgcttctgtctggggctgattagatcttttatagataccaaagcatcatgtataacatgcaattatagacatgtaagaagttcaacatctagttttatgcaaaaatgtgaacttacatctggaattaacctgtaaaatgattagcaaaaaattagttcattttctggaacgaccaccttaattattgaattacatctccttaatgaatttagaggtggcttgctgcaaatttaattttttataagattttcttgtggaaaatctgctaacatggactcaacaccagatttattatcccacatgaaattatgctgacaagagaaatttatttttagttttttggatttagcaataatatgatggtcttttataaatcctgtgtgcaatgataattagcatgagttccatcttgtgctgacatctgtgttccaggggtattatttgaatgatgttgtctttatcttttcttctgatccccgagcacattttcttaagctcaagaatgatttcagtgatgctgccaccataatgctttacatttatgagggagttggtgacattgtcttcactcacttcctgattgattctctggggaagacgaggctcaatcgtgcttgcttgattccacattttttgcatgagtgccttctcaacgagcagtacaggtaccattgtttcagcaagcttccaggggcatctttcgaaccacttcccaagcctattttcttgaccttggctcagcccttcatgaattagttctttatgctcaaatatgattctagtgatctggtcctcatgctgccacaataatcctcaacatgtaggagggagatggtaacattgtttacactcacttcctgcttgatactttggttccaaaattttggataagtgccttccaaaagggttatagcattgatgaacttgatatagttcttctctttaagatttcactgcctatcactaggggctttaaaaatgtgtgagtgaaaattgaattctagttgctgggtcaattcttgatcatcattaacactaagcaatcttgagctgggagggtactgttgcaatttggaacttgcccgatggcaaaaattaagtcacctttccaaaggtaatatattaaaggtaactttgataactttgctattggtttattatataagaggaaggccgcatgatcttacatctagtcttcgagtatacatcttccataaaatgctaattaaattgataggctcctaagacccactgttaatttagaaacccggtctgagcttattttttagttgaatacaaacaaatctggagttgtgtttctcacatcctctttgtcagacagccagtcaaacacccaataagttgaccaaaaaactagttgataattgttgcagcttttttgtacacaaatgttagatgatgttgggaacagtttatgacctttaaatggcatttggaaggatatttgatcacatcaaagtggtggctgtttgaccaagagtttgacgaagtgggtgtcagaaagcatttcacagagatcttaattattttgaatctgtacttttcctgtatttatcttctgcacaccatgggtcactcatgaatcatgatgttttaccgaaaccttttacttcagcttgaattctcacccattctgaattttctgcaggtgataagtaacggtgaatataagagtgctgtgcatcgagctgttgtcaatgcccatcatccccggttatctgttgccacattttatgatccatgtaagaccaggaaaatatatcctgctatgcagctaatcaccaagcagtctccactaaagtaccgagaggttctttatggggactatgtctcgtcatggtacagcaaaggtccagaaggcaagcgcaatattgatgctcttttaattaaccagtaatgcatcattcttatattgtgattggtctatgaactcctaagctcgcccaagttgagatgtgctctgtaatgaaaacatgtatgccaataaggattcttggtggaagatgtctatcaagattatagccttgaacaaaaaggtacgtaactttgaaagcaacaagaaaaaggattgtgaataggtatgatttttgtctcatttcacacatatctgcatcttttggtgttggaaatttatctgtataaatcagcaagcattctatggaaggtttagattatgggatttgact

SEQ ID NO: 36 - DNA, 1718 bp, Musa acuminata
  source 1..1718: mol_type = genomic DNA
agaagactgagtcaagtaccaaaagataagcttcttggtaagcttattgctagacagtaatggtggcgaagcttctctctctataagtgttgtcgaagctgctacctgcccaaaccagccgagctgagaggtgttagtcttcgtacgcggtgtgtgcgcgcttgcttgcttcgcgagatggcgaccccgagctttcagcgtctgggaacgtccatcgacgtaccgaacgtccaagctcttgcagcttccatcgcaaacccggctgacgtccctcctcgatacgtcaggccggaagccaaggctgatcccgtcgttagcgacggcgacagcgagcttccggtcatcgatttctccaggctcctccatcgccgtttctctagggaagagtctgctaagctccaccatgcctgtgcagactggggcttcttccaggtcagtcgatctacggatcgaaatcgtgtgatcgatagctgcaacataacaatcgttgatgctaattaacagttgataaatcacggagttcccgatcaagcgatggagaagatgaaggctgatatagtagaattctttaagcttcccttggaacagaagaaggcatttgcgcagttgccgaacagcttggaaggttacggccaaatcttcgtcgtgtctgacgaccaagagctggactgggcggacattatgtacctcataactcgaccactccagtcgaggaacatcgatctctggccagctcaacctctcactttcaggtttatctcgacttcttgtgctgtcatctactcagcggttcagctacgtacttattacgtacatgacgtcctttgctgccgcttcatgccgtcagagactctctctcttgctactccatggagctgaagggcgtggcaggaactttgctggaggtgatggcgaagaatctgggggtcgcaccggaggagttctctactatatttcaggaccaaccgcagggagtgaggatcaactattatcccccatgtccaagggctgacgaggtgttgggcatctcgccacacacggacggcagcggcttgacgttgctcctacaggtgaacgacgttgtaggactccagatcaggaagggggggaattggttcccggtgaagccactccccggcgctctcatcgctaacatcggtgatatcatcgaggtcattaactcgactcaaattagtcagaatcaacatatatcaatcatgtccgatactaattcaattcaaaaataaattatgtttatagattacgagattctctcaatatttattaatgtaaaattattattattttttttttcaatctcttctataaatattttctaacaaaaacaaaagacttttggaatagatattgagcaacggcgtatacaaaagcgtcgagcatcgggctataataaatgccaagaaagagcgtcactcgatcgctaccttccatgggccaagagaagatttgatggttggtcctctctcagagatcgtgaaggagtgcaagccgaagtatgtgtcgatgagttacaaagagttcatgaaaacttacttctccgcaaaactggaagggaggagcctcatggaaagcctcaagctatagaagtctctaatgttagaaagttcatagtgtgttgcttgaacttgataataagtatgttttgggataatgttatataagcatcgaatctttgtatgtttaaagtgtattgactt

SEQ ID NO: 37 - DNA, 3586 bp, Musa acuminata
  source 1..3586: mol_type = genomic DNA
tctgcgcatcgcgtttccccgttcgacctcgcacaaccttctctcgctcgctcgcgcgctctcccgtttcccgctccgtccgatggcagaccaacttctctctgcggtctccgactacgtctccatcccggagagttacgtccgcccggagtcgcagaggcctcgcctcaacgaagtgatccgaggagccaacatccccaccatcgatctcggctcagaggatgagctccaaatcatagcgcaagtcgccgacgcctgccggtctttcggcttcttccaggtacgtcgtcaggtactccatgatgctgtgtatcatcgtggtcatgtatacgtatacgtacacaggtggtgaaccacggagtgccgctggagtcgatgcagaagatgatggcagtggcttcggagttcttccgcctccctcccgaggagaaggcgaagcactactcggacgacccagcaaagaagatgaggctgtcgacgagcttcaacatcaagaaggagacagtccgcaactggagagactatctgcggctccattgctatccgctggaggagttcgtgcctggttggccttccaatcccgcttcatttaggcaagatttcactcccatctctctctctctctctctctctccatctattgtcaagaactttatagactattatttgttgaccggaagctggagaagaccttccacccagtttttgtcagcgtcatgttgcccgtctacatttcgcagatgagatcagggtgagaaccttattcctcaaaaaataggacaagaagatgcgtccaagatatataaaccccacaaaagatactaatcatatataggatggtccaaatctgagattcgatgcgcatctaatacctgcagacactctgcacacggagatcacgccatgcaaattattggcagcaagtgatgactgatgagctcactttatattattaccttcaggactgcatgtaggagagaagcacaacaacagacccctctttccctggtttaagccttgcatgttgcgactgttcatgcattactatgaaacatcgactctgtcaagggaaggacgaatcaattatggatacctgcttgaattatgtagcttgaaataaggaatttctttgtcaatcttggagtaggaccaatgacatatatctcgatcaatgacacatctgctcaaagcactagctgatccccttcaatgtttatccacatagaggaaaagtcctctccaacttgttgaagatgtagaaaatggtccctctttcttgtaaatggagacttctcacctaaaacgtatactcgatgtttttcttctctttgacaagtacaaaaggggcagacatatcaaagatgaaagatgagagagaagacaaggaagaacgaacagtaacccttttctttttttctctgagggtggcaaatgtaggtcatttttgcaccttgtatctattaactattcatcaacgcccttctggtcctcgattatcatgtgatagggaaatgaaagatgtagcggacagataagcatacatacatttactatcagaggctcagacacagcatgtgaagtcacatgaaaggttcaaagcaaacagttggatcataagctactgggtgcatcacagatctataataggtggtatatttaatctttgctcagagattataagctctttgctttgttcatagatcaagtcgttctccatgtcatgaagaacttaatcgttctgcctttctctctgtctcagggatgtggttagcacttactgcagggaagtccgtcgactagggtttcgactcctgcgagcaatatcgctgagccttgagctggaggaaggctacatggcgaaggtgcttggggagcaggagcagcatatggccgtaaactactacccaaagtgcccagagccggagctcacctacggcttacaggctcacaccgaccccaacgccctcaccgtcctgcttcaggacccaaacgtcgctgggttgcaggttctcaaggacggcaaatggatcgctgtcaatccgcaacccgacgcgttggtcatcaacatcggtgaccaactacaggtaccgatgcttttgacgaactctggccttcgttgagatctgctctgcttgtccttcaaatatactctacatataatactaattttcctaccgaggatggtcaaatagtcagacgaatacggtcgaaagcatggaaaagaagaaacattgttgttagtgctttcagccatttggtatacgtctccatctaaggatcaaagcttagttgttgccattgggtactttctgcaactgggggaggaagggtaaaagcatcacaaacacatgcatgcttatttcctttggcgaacatggacgaagagtactttttcctcctagtcttgtgatctaacgttgggcttgaaagaataggtgggtttttccaagctcacaccatgggcggtactatagtcaatggtcagcatggtcatttccttgcccgccactgcttccaagccaaaatctcttgttccaatgtgggtcttctttgaccagcatttgattttacttgcattcttaaaagccactgtacgttgggaggtagcagatccccgagtcaagaacatgattagttcttgaccacactggaaaacaatgggtactgcacgccgtggaatcctggtaaacttgatggatgcttggtctttgtgctcatctgtcctttcgtggtcatcgtgctcatcttggaagtggctatgatcctacaattgacctccatcttttgtgaactagtcttccactgtcacgaaacaatctcctgagcatcttcaaaagagatatagactgctttggttccatgtatgagatcagctgtcagttgaacaggtgagcggtagctgatgccaactgctcttgatcatgtttgtcgatgccctcttcttcttccaattgtcgagcggcttcttcttttcatggattgatcgagaagaaggtgacgtttgtccattggcgcgactatgttgatgcaggcactgagtaacggaaggtacaggagcgtgtggcatcgagcggtggtcaactcggagagggagaggatatcggtggcgtcgttcctctgccccagcagcagcgtggtgatcagcccgccggagaagctcgtcggcgaccgggctcggcccgtgtaccggacctacacctacgacgagtactacaagaagttctggagcaggaacctggacgacgaccattgcttgaagctcttcgagtgctaatggcttgccgacgagggaggaggcatcccacgcgacccaggatggcggcctacgttgctggtatcgtggccacatcagcaagtacaccagatgatctggcatgctgcttcttgacatgcctccgcgctgtccacaataagctatggacgtattaaatttttggtatacggaggcaaatgcatagtgctcatacgaagctttcaggcatggcaataatgtctcttccttgcaaatagaaccgtcatcagtatctttacgttgcttgtaagtatgatataaataaatggtttgctggagattctgcgaaggaaa

SEQ ID NO: 38 - DNA, 5803 bp, Musa acuminata
  source 1..5803: mol_type = genomic DNA
cctgagaaccgtcccatggccgaccggctcctctccactgtccctcaccaccacagcctcccggaaaactacatccggccggaatctcaaaggcctcgcctcgccgaagtcatcagcgacgcccacgtccccgccgtcgatctgagctcacccgataagtctcatgtgatcgctcaaatcgccgacgcctgccgatcgtacggcttcttccaggtgtctttccgtgagcaggcaacgtaaggtacttcttctatgttggaccccgtgttactggcttgtggtctttataggtgttgaaccatggagtgccagttgagctgatggtgaagatgatggtgatcgctctggaattcttccgcctccctccggaagagaaggcgaagcactactcggatgacccggccaggaagatgaggctgtcaacaagctttaacatccggaaggagacggtccataattggagagactatcttcgtctccattgctaccctctggaggactacgtgcccgagtggccttccaatccttcttcattcaagtgagaactaagctcccctcctcctgcatgctcttcctctcttcttccccctcgctttgcatggtgaaccatgtcagcaaaggatttcttagctacatggtgccaaacaagacctgtttcacctagtaacctatctagcttgaaggtcttatttatcctttcttttctcctttcgagaaaagcaataatagtctcagatgttcatctgcagctaaaagcagcgagttttgaaccctcatatatgccattagcaacctattttgaggaagcggtatgcggccattagctcttgatatataatataatctttgtgtgcaaacctctccttatgtgtcagtcttgtaggagagattgtgtagaatccttaactattctttatcttgaatattattcccgataaaaagcaagaacgaaccatggttacaagtcttctatgaggaacctttgtatcatctacatcatgattctgattctgatagaatgcacattgtcattgacatgacatgctttgataatctaacaaaaggacatcagactatatagtacttttaatagtggacatgaccgacgtcgggcttatcgagataaattaaatcgtgttggaatatatgtcctaatctgatgtatctgcacaaactgtgaagatggactattgcggcatcttgcgaggaatttgatgtgcttggctttgtcagggaagtggccagcgcttactgtaaggaagtccgtcaactaggttttcggctcctgggagcaatatctctaagcttagggctggaggagaagtacatggaagaggttctgggggagcaagaacaacacatggccgtcaactactatcccaagtgccctcagccgcagctcacatatggtctgccaccccacacggatcccaatgctctcacaattctgcttcaggatcccgacgtctctggcttgcaggttctcaaacacggccaatggatcgcggtgcatccccaaccccacgccttcgtcatcaacatcggcgaccagctgcaggtgacagcgcctccctcatcctctcttgcacttctatttttagtttttgaattacataaatgaaagaagagatcatataaatgcaatttttcttaaatagtaaccatttttaaaataacagcatcaagatattagctcagatcaaataggaaaaaaaaataagatcgaagtatatatatatatatatatatatatatatatatatatatattaaagatataaaatactaatttaaatcaagaaatccttatctttaaaagtctatctaatcaacttatttaaaggacaaaagataagaaacttaaaatcatccaaaagataatactttaaatcttagcatttctctttaaattataattttaaatctggggcgacatcacatgtgcaatagaagaacaaaaaataaaaatatcaaaatttttcatagaaaagaaggtttcatcgtcgtatgaagattggtgcgtaaaaattcacggaactgaaaaaccacgcgtgttaagggatgtgtgttacctaggaagatcgtatatccttgaaaacgtatagatctatgagagaggatgaaggaggttaattgtctatctctctagcggtgtttcatatggtatgagctatgaagacgctcctcaaatcgctgctcaaatctattcactatgtgcaccatacaatcaagaagggggcaacccttcttattgttcacatgttaataggggctattgaccgaaaaggagagagagagagagagagagagagagagagagagaagaataggaggtgaaagccaaaaggggtttagcttatagccctttggtttcctcctatttatagaagtcatctgtcaacttaactctaatggatcatactatattgggtattggatctccatccaattacccaagcttcttagattaatgagtctttatccaatattctcttattggatatcatctataggattgaataatttatatgcttattagatatccaataacataataagataggggctctagtgaatatctcatatccgaacacctactcgtcataacacataccatatatgtaaccatctaaccttaatatcaagttggcgaatcatacctatcagaactccttctgactcagtaaattattatctccataataattcacttgactcatcgactacggatatattataccactacgtcgtagtctctatctgatataggagaatctaatctattggatatatctgtccttagttcccatatatcgatagtctctcatctatctaatatctcatagatcatattccgagcatggtgctgtcaaactcatacgatgtctactcaagtcacgctctaatcggattctcccaaagaactctttctctttcaatccgaatgaccttagctagggatttgcctgagcaagaatacatgagatatttctctcataacataaagagtggatcctctatcaacactcaatagcctttgtaaggttggctgtcactccctatgatcgactgtactagaattggaactttaaagtctataagtttgatataaaagagtggaatactcatacaaaacatccttagtatctcaagtttaaggatcatatacactactaagataacggaatcactatatgacaatatggtatcattaaccatctagcattttgtgagcagatcaatcagtgaactcattctccaataagtacctacgcattatccctagtgtcccacacgacgagaccagttgcctctaatacttttatttaagttatgctttatcttttagacttatttgtaagttttaacgcatgatctcaagttttatttttatctagagtttttatttcttcatcgatgatatcctcctactccctaacaccttttttcttcattaaaataaataggtttaaaagaaataatgacttatgctacattatctccatctctataacatgctggcttggtaattatttttttatcttctcaatgttaaaattttcacttcatgaacatcattactccctcgtttactttgccccaccattagtgacaaagaaataatagaagtagatatatacaaagaagaaaataagtgaaaattataagagtattaaatgataaaggagacttaatcatacgttttaaatatatatcatttttactattgtgattgatatttaaaaaaaactatttatggaggataataagaagaaactttatcaaacataatatctcgagataccacatacttatttgtttatggatccatgcatttcaatctttctttctttcatcatagtcaataaagataattttttggtcttaataaagataatgtgaatatagcacaaagaaccaaatactttataatgaataacgtttaatttcataccaaacatgagcctatatgaataatttagattaattggattgaaaggaacttgattaataatataagttacttaagtcatctttctacttataactctttctttacaaaatagatccaagtaaatcttataaaatcattaataaagaaaagcatataataaaaatttgaataagataaagtttgagtaaggcttgttagattgatgtgaacaagctttaagagaaatttacacctcgaaaataatatatcaaaaggttagttgtgtgctttgtgatattgacaaccttgataaactttattatggttaaaagtagtaatatggttaactagactttctacatcataatttttaatttgaaaaaatttatatgaccaagtctagcatgttagatgttgataaaatatataaatctttgacccttttattattgtgtataacatctatatttaattattttatattataaaaaaacttaacttttttatgatcaataagaatataatttctaacatcaactacatttgcagtagaaaaataaaatttcttcacatgatacacattctttaatgtaatagaattattatccttatctgagattataatattaccttcatgatgtctccatcttcccttaggagataaagactcccaataaattctctagatcttatcgttggactgatcgagaagctcgatactaaattcaccaacttgactattataatttataatcgaaaaaaggtcatcatcttgaaatatagattatcactattatggttctgataccatgtaaagaaaatgagagatcatatacaagtacaatcagttcttaaataataataataagaatcaaataaaagaagaagaaatcaagatgtactaaaaacagaaaagctatattgaacttctcaaaaagaaaaatataaaaatatttacaagatattgaactattttttgacttgagttgtatagacttgaacacttaaaagacttaaataaatttacatatataggcatcatctatttataggtgtagaataaaaatttaaatcaagagattctcatttttacaagttcatctaatcaatttatttaaaagataaaaaataaaaaatattaaaattttctaaaatataatactttaaatcttaagattacacctcatggcttcccaattcacttcactatattttggtcatcttgcactcgattctttgtttataaagaatctattgatgcattacaaattagacttttccttagtccgacatatgaaaagaaatgcatgcatcttgtagtagcatacactaaccactataatgttgtggaatcatcctgttgattttatgttaagtgacctttggattttcttttagtttccaagttcttctctctatctaacaacataatcgatgccttgttatgaaagaggcagaaaagctctgcatgaacaaaggtttcactttgccactggagccatatttccgtaagtttcatattaatggctatatcattgcaggcattgagtaatggtaggtataagagtgtttggcaccgagctgtggtgaactcagagaaagagaggatgtcaatagcatcattcctctgtccctgtaactgcgccatcattagccctccggagaagctcatcagcgaggcatctccggccatgtacaggagctacacctacgaggagtactacaagaagttttggagcagaaacttggatgacgagcactgcttggaggttttccgaagctaaggtgtatctatcaatgaacactgtgttcgttggacaatgccaccctagttagtaatgttgggaaagaaggcatgaggctaaaacaa

SEQ ID NO: 39 - DNA, 2099 bp, Musa acuminata
  source 1..2099: mol_type = genomic DNA
cctccgccgcttctcaagtccgaccaccacaaccactttctttgctgcttcctcagcaaagaccgcaggatggaggtggagagggtgcaggccatcgcgtccctgagcgtggccaccaacgacataccgccggagttcgtgaggtcggagcacgagcagccgggtatcaccacgtaccgcggcccggtcccggagatcccggtgatcgacctcgaagacggggacgaaggccgggtgacgcgcgccatcgcggaggccagccaggagtggggcatcttccagctggtgaaccacggcatccccggggaggtgatccgggcgctgcagcgcgtgggcagggagttcttcgagctgccaccggaggagaaggagaagtacgcggcggcgccggggagcctccagggctacggaaccaagctgcagaaggacttggaaggcaagaaggcgtgggtggacttcctcttccacaacatctggccgccgacgcacgtcgaccaccgcgcatggccggagaatccagtggattacaggtgcccgctcctacctctccttgcacgacactacgcttggtccaatattgtctaatatactgttctctcgcttatctcatgcagcacttatatgtgtcaccagcacttgtatggtctctctcttctgcctatacgacactacctttccttcctctttctaggactgtttaatttgatgtattataaatctataacccaatttagattgtattcttaaatctttttagatctctaataatactttcgatatttttgttagaagtaaaatctttaattatgaggaagtgtgaggactctaatttttgcgtgtactttatagatataatatttcaagtagactctctctttaatataatattaaaaatattttatctaattcaacaaaagtcaattatttgtttaaagttgatagaaatagattaatcttagcataattaattattacgagaaaaattcttttaaacaccaaatcaaaatcattatctctatgtatatttcttagaatttagatctaagacacttccctatctcctgtcttcatgttaaatttgaatatatatatatatatatatatatatatatatatatatatatatatatatatatatatatatatatataaaatcatttctgtggaatatttgtcttaaacaccattcctgtgggggggagtgacatgtcacgaggaactcaggtttcgtcttctcctctcacgttaagtattcatccacttccatcacattaaattatgtgcaggagagttcatctaacctaattatttcaggaaggcaaatgaggagtacgccaaacatttggtgggattggtggagaagatgttggtaagcctgtccaagggactggggctggaggccgacgtcctcaagcacgcagtgggaggggacgacttggagttcctcctcaagatcaactactacccgccgtgcccgagacccgacctcgccctcggcgtggtggctcacaccgacatgtccgccatcaccatcctgatccccaacgacgtccccggcctccaggtcttcaaggacgaccactggttcgacgccaagtacgtccccgacgccatcatcgtccacatcggggaccagatcgaggtatgcagacctcaaactatgcttcctcatcaatttcatgtgctgatgacgagtggttgcagaaactgagcaacggcaggtacaagagcgtgctgcaccggacgacggtgaacaaggagaaggcgaggatgtcgtggcctgtgttctgctccccgccgggcgagacggtcattgggcctctgccgcagctcgtcagcgacgaacagcccgctcagtacaagacgaagaagtacaaggactatgctttctgcaagctgaacaagcttccgcagtgaggtcgcaccgggttcttcttgcatgacggtattgctgtactttgccttatgtgtgggtcccttttaagctcatatagtggtctctgtccactttgagttggcataactccgttggagcagaaggtggatcccgctccatccttcttatctaataaacgaatatttggatgtaagccatcagc

SEQ ID NO: 40 - DNA, 1483 bp, Musa acuminata
  source 1..1483: mol_type = genomic DNA
gcaacctcgaccttcctcggctgtccaagtattctctctctctctctctctctagatctgtgcctcccttccatggccgaccaacttctctccaccgctcctgactaccatagcctcccggagaactacatccggccggaggatcaaagacctgttctcactgaagtcgtcagcgacgcccacatccccgccatcgatatgggggctcccgataggtctcacgttgtctctcaaatcggccatgcctgccgatcttacggcttcttccaggtctcttcccacacacatacatcacaggattctaccgtgttcagacttgggagtgcgctgtatgattactggcttatgttcgtgtataggtggtgaaccatggagtgccagttgagctgatgctgaggttgctggtggtcgctcgagaatttttccacctccctccgacggagaaggccaagctctactcggatgatccaaccaagaaggtaaggctgtcaacaagctccaacatccggaaggagacgatccgtaattggcgagactatcttcgtatccattgctaccctctcgaggagtacgtgccggagtggccttgtgatccttcttctttcaagtgagaactaagattaattgagtgttctcctcctcctgctctgtcctctcttcttcctcaaatgtgcatgacgtgctctatgggcttagtactttactctcatctaagaactttcaccaacaacagttgaagtattatcaatttaatacaccctaaagttgcgatgactttatattgttctttggcagggaagtcgtcagcgcgtactgcaaggaagtccgtcaactgggccttcgtctcctggaagcaatatctctgagcttaggtctggaggaggactgcttggtgaaggcgctgggcgagcaaggacagcacatggccataaactactaccccaggtgcccgcagccgcagctcacatacggtctgccagcccacacggatccgaatgctctcacaattctactgccggatccggacgtggctggcttgcaggttcttaaagatggccgatggatcgccgtagatccccttgcccacgcatttgtcatcaacatcggcgatcagctacaggtgaccacccttggcttgctgatgatccatatattcttgcgttgccattagctttaatggttatgtcgttgcaggcgttgaccaatggtaagtacaagagtgttttgcaccgagctgtggtaaacccagagaaggaaaggatatcggtggcatcatttctctgtccgtgtaactatgcaatcatcagccctccagagaggctcatcagcgagggatctccggccatgtacaggagctacacttacgaggagtactacaagaagttttggagcaggaacttggatgaggagccctgcttagagctgttccaaagctaattgtacaaacgaagggacagccgaaaccaaataaaagtatattttg

SEQ ID NO: 41 - DNA, 2049 bp, Musa acuminata
  source 1..2049: mol_type = genomic DNA
ctgaatggttggttacttcgtccgtccgtcctcgccctacctatctctaagtcccacacggtcctcatgtctctcctatgctctccgtcgtgcttcgtccatggcagaccagcttctctccacagtaacccaccacggctccctgccggagacctacgtccgtccggagtcgcaaaggcctcacctaaatgaagtcctccgcgacgccgacgtccccaccatcgatctcggctcaacggacttgtcgcagaccgtagcgcaagtcgccgacgcctgcagcacctacggcttctttcaggtgcatgtccagcttctgcaacctgggacaaacctactgctgcgtgcttcaactgttccttgctgtatatgtgtgtgtgcaggtggtgaaccatggagtgccgatcgagttgatgctgaagatgatggcggtggctttggagttctttcgcctcccttccgaagagaaggcgaagctctactccgatgaccctgccaagaagatgaggctgtcgacgagcttcaacgtccggaaggagaagttccgcaactggagggactatctccggctccattgttatcctctcgaggagttcgtgcctggttggccttccaatccctcttcatttaagtaagtcttctcccaattttttctcttcaggaaagtccaagaatatacatattatacatatatatattcctcttcctctttcttcttctccttgcatctcttaggggttgattccagctccatatctgtggcatatgattcatcaatagcaaggaaaggataagataatcctggagacctgcttcttttagccgatcgtcatattgggataggaatcttgacatgtaagccaccaccaaaatctcctgagattttgatagagtccaattgttttttgatgtgatgagcttagaagcatagaaaaatgtggaactggtccactgaatggaatcttctttcacctaaagaagattccaatgtttcttttttcttttccttttgatcggtacaacatgcagaaatttcaaagattaatttcaactctcttaaggagaaaaagaaaagaaaatgccaataatgatcaaccagattatatgacttcacccgaagcaacacagttcattttgtactgttatgttgtcagggaagtggtcagcagttactgcagggaagtccgtcaactggggtttcgactcctcggactaatatcgatcggcctgggactggaggaggactacatggcgacggtgctcggcgagcaagagcagcatatggccgtaaactactacccaaagtgcccggcgccggagctcacgtacggtttgcaggcgcacaccgacccgaacgccctcactctccttcttcaggacccagacgtggccgggcttcaggttcgtaaggacggcaagtggatcgctgtcaatccccaacccaacgcattcgtcgtcaacattggtgaccagcttcaggtatcggcatatacttctgctgctgattgtttctggagttgtttgcataggttatgcaatcatcaagtcttgccgtcccgaaaagctgatgaaacatggtcgacatggattacgtcgatgcatgcaggcactgagtaatggaagataccggagcgtttggcatcgggctgtggtcaacgcggacaaagagaggatatcggtggcgtcgttcctttgtccctgcaacaatgccatcatcagccctccggagaagctcgtcgccgacggatctccggccatgtacaggagctacacctacgacgagtactacaagaagttctggagcagaaacctggatgacgagcactgcttgcagctcttcagaagctaatgcctaatgctgctgcccgtggcatgcaacaggatgagtgctctacgtggcaaccttgctgatgtggacatctcggattggtcaaaagtgggacgatttcatgacatgtctcggcagcgtttcggcttttgtgtagtaagacaaataatgtttgaccgtattttgacttcaataaactaaaacattgcaagggaataataaat

SEQ ID NO: 42 - DNA, 1658 bp, Musa acuminata
  source 1..1658: mol_type = genomic DNA
gaagcaagacaaccaagcgaagcttctctctctataaatgttgtcgaagctgctacctgaccaaaccaaccgagctgagaggtgttagtcttcgttaaggggtgtgtgtgtgcgcgcgcttgcttcgcgagatggccaaatcgagctttcagcgtatgggatcgtccattcacgtcccgagcgtccaagctcttgcagcttccatcgcaaacccggctgatgtccctcctcgattcgtcaggccggaagccaaggctgatcccgtcgctagcgacggtgaaagcgagcttccggtcatcgatttctccaggctcctccatcaccgtttctctcgggaagagtctgctaagctccaccacgcctgtgcagactggggcttcttccaggtcagtcgatctacggatcaaaaccgtgtgatcgatagctgcaacataacaaatcgttgatgctaacttacagttgataaatcacggagttcccgatcaagcgatggaaaagatgaaggccgatatagcagaattctttaagcttcccttggaagagaagaaggcatttgcgcagttgccgaacagcttggaaggttacggccaagccttcgtcgtgtctgacgaccaagagctggactgggcggacatgctgtacctcataactcgaccactccagtcgaggaacatcgatctctggccagcacaacctttcactttcaggtttatctcgatttcttgtgctgtcatctactcagcggttcagctacgtacttattacgtacatgacgtcctttgctgccgcttcatgccgtcagagactctctctcttgctactccatggagctgaagagcgtggcaggaactttgctggaggtgatggcgaagaatctgggggtcgcaccggaggagttctctactatatttcaggaccaaccgcagggagtgaggatcaactattatcccccatgtccaagggctgacgaggtgttgggcctctcgccacacacggacggcagcggcttgacgttgctcctacaggtgaacgacgttgaaggactccatatcaggaagggggggaattggttcccggtgaagccactccccggcgctctcatcgctaacatcggtgatatcatcgaggtcattaactcgactcaaactagtcaaaattagcaatcaagtgcgatactaattcaattcaaaaaaaagttgtttatctcaatatttactaatgtaaaattattattattatttttttaatcttttcttacgtataaattattttctaacaaaaacaaaagactttcggaatagatattgagcaacggtgtatacaaaagcatcgagcatcgggcgataataaacgccaaggaagagcgcctctcgatcgctaccttccatgggccaagagaagattcggtgattggtcctcttgagatcgtgaagggatacaagccgaagtatgtttcgatgagctacaaagagttcatgaaagcttacttctccacaaaactggaagggaggagacttatggaaagcctcaagttataaaagtctctaatgttagaaagttaatggtgtgttgcttgaacttaataataagtgtgtttcgggataatgctatctactttatcgaagcatcaaataaacacctagtgttgtgtatatgaa

SEQ ID NO: 43 - DNA, 3064 bp, Musa acuminata
  source 1..3064: mol_type = genomic DNA
tccgccttctccctttatttgtgcagcgtctcgaagctccctttcgatacctctgtctatctcatggcggatcagctcctctccaccgtaacttaccacgagacccttccggagaactacgtaaggccagagtctcaaagacctcgtctcacacaggtcatcagcgacgcaaacatccccatcatcgatctcggttcaccggataagtcccgaatcatctcccagatagggaaagcctgccaatcctatggcttcttccaggtcattgaattccgactacccagcttcttcctttcctcctcaactgtatgctgagtatttcccgggttattcgtttgtaggttgtgaaccatggaatcgatactgaattgatggtgaagatgatggctattagtctggaattcttccgtctacctcccgaggagaaggcgaagctctactccgatgacccggccaagaaaatgaggctctccacgagctttaatgtcagaaaggaggcggtacacaactggagggactacctccggcttcactgctatcctctggaggaatacgttcccggctggccttctaatccctcttcattcaagtaagttattcgtgcttctcctcctcttcttctctttagtcggacagtaatagcataagaatagtcaaataatttgagtatgtactgaaaaaaaaaggtgataataagaataataataataaataaagcattgatgtaaagactgctggaatacccatcgaatctctatgtagcgattggacaggtgcatattaccagtatgcttgattcgataggctcgcatcttgatgctggttaagaatctgatgctgccagagcatgatgcatgtataggagaaacactccagttcccttaagtcgtcactagaatttggttctttgacgagagtagcagtgtgcatgaagccattagctgctgatgatgatggattatggttgatcacttggaattaatacttcatgtctctggatcttatgattggtcattgtcgtagaagacaaacatggctggaaaatataatctgctgaggtaagaacattctagtgggggaatcttcatcgtgtgaggcagtaccaaaccttccttgtgggatatttttagatttttttataggactgacagtaacatggttatctatacggagatttcataacatggactaataaatcaagggaaaacacaaggtttcatgaaagtttgtggaagacaagatccgggtcagtacgaacctctggtcagaaaataggtgcactcataaaagcaccattcccggagtcatacaagacatcccacttagagcagtgcatttaaatatggggaaacagatgactcaaatcctgcatgtgcaggcacatgttcacagtcgcagaacgtatgcatctgcaaatgggtctgcaataaaagttctttaactggatggtcccgtttcttgatgattaagtttgaagagattgctgcgttgttctttctgttgtgtgtgttccagggaagtggtgagcacctactgtaaggaagttcgtcgactgggatttcggctccttggagcattatcattgagcttaggtttggaggaggagtacatcgaacgggtgctgggacagcaggagcagcatatggccatcaactactacccaaggtgcccggaaccggagctcacatatggcctgcccgcacacactgatccaaatgccctcaccattcttctccagcagcccaacgtggctggcttgcaggttctcaaggacggcaaatggatcgcagtggaacccagaccgaatgcgtttgtgatcaacatcggtgaccaactacaggtgattgctaatcacacactcgttctatctcgttaggagatcctgatacctaaaaacaaaggaaaagcacttctttcttgcacgaatcaaggaaaagcaccttattttttgatggtgttaaggaccatggtttgtagtttagagttgccctttgaacgccatggtcagacgcactggcccatttcctcgttttgctgagcttgcctgccatgccctgcacatgacagcgtgcagctgagctttggcaattatcccaatcctgcccatgtctaagtagcaataatgtttttccagcaaccagaccgcttgatcccagtctctgtcttcgttttctactcacagacatatgcaactcttccagaggcattcacaatgtttgccgatagcattgtgggcttaggcgatcttgcactttatatattaaatatgtaaatcggttcttgtgctctactttcagatttccatttgtttatgttcaattactacttttcttttcctccaatatcgtcctcctagtttgtgcatcagagaagcactaaatctatgatgctgctcccatctcacatatgatatcagcctatcggcttaaagtaaaagtgtgatgaagctttggaaaagctgcagacgattaaatattttcacgcaggcattaagcaacgccagattcaagagcgtttggcaccgagctgtagtcaactcggacaccgaaaggatgtctgtggcgtccttcctctgtccatgcaacaccgcgatcattagccctccggagaagctccttgccgagggatcaccagcggtctacaggagctacacatacgacgagtactacaacaagttttggagcagaaacctggatgacgaacattgcttggagcttttcaaaggggagaagagccaatcaggtggactgagcggcccctgcaaaagctcgacatgatgtgacatcacacggacagtgcttcttcgtgatgctggttgattccgttcatcatgtggagcacaaattatttgcggagactctcgtgttgtccacgatcgacagtgaggagagttcggtggtctgccctcttattgatttatttattcctgctttgccatgttacctttcgctaccaaagcactcgacttgtctgcaccatggagttcggagctggcccgccgtctccatttcttaaaattggctctgtaatccagtaactgcttgtatcattgttttgttctctc

SEQ ID NO: 44 - DNA, 594 bp, Musa acuminata
  source 1..594: mol_type = genomic DNA
cccccgatgcgccactccatcgtcgtcaacctcggggatcagcttgaggtttgcgatctccacccggtctgcgccactacacgcttaaacagcattaacactggattcttccgtgcaggtcatcacgaatggcaagtacaagagcgtgttgcaccgggtggtggcgcagacggacggcaacaggatgtccatcgcctcgttctacaacccgggcagcgacgccgtcgtcttcccggctccctccctggtgcagaaggaagccgagaaggacgacgtggcggcggtgtatcccaggtttgtgttcgaggattacatgaagctctacgtgatacagaagtttcaggccaaggaaccgagatttgaagccatgaaagccacggctcttcccattcctacatcttaagaacatcaacagtcgatcctcatccaattcctgcatctcaataatatgtcatcgtggaagctaccagtatgcagtaagaacttagcaaaggtcatgtaacgtaagcaccgttatgccagtgagagttcctaggcatgtgttatcttaaattagactttttatctttgaggaaataagtggagcactgtaaa

SEQ ID NO: 45 - RNA, 23 nt, synthetic construct
  modified_base 4: mod_base = OTHER; note = thymine
  modified_base 6: mod_base = OTHER; note = thymine
  modified_base 11: mod_base = OTHER; note = thymine
  modified_base 17..18: mod_base = OTHER; note = thymine
  misc_feature 1..23: note = sgRNA sequence
  source 1..23: mol_type = other RNA
gactctaagatcagggttaaagg

SEQ ID NO: 46 - RNA, 23 nt, synthetic construct
  modified_base 6: mod_base = OTHER; note = thymine
  modified_base 11: mod_base = OTHER; note = thymine
  modified_base 17..18: mod_base = OTHER; note = thymine
  misc_feature 1..23: note = sgRNA sequence
  source 1..23: mol_type = other RNA
gcagctaacatcagggttaaagg

SEQ ID NO: 47 - RNA, 23 nt, synthetic construct
  modified_base 11: mod_base = OTHER; note = thymine
  modified_base 22: mod_base = OTHER; note = thymine
  misc_feature 1..23: note = sgRNA sequence
  source 1..23: mol_type = other RNA
ccaccggagctcaggaaaccatc

SEQ ID NO: 48 - RNA, 23 nt, synthetic construct
  modified_base 11..12: mod_base = OTHER; note = thymine
  modified_base 14: mod_base = OTHER; note = thymine
  modified_base 17: mod_base = OTHER; note = thymine
  misc_feature 1..23: note = sgRNA sequence
  source 1..23: mol_type = other RNA
ccggagcgcattgtaatgagcgg

SEQ ID NO: 49 - RNA, 23 nt, synthetic construct
  modified_base 1..2: mod_base = OTHER; note = thymine
  modified_base 5: mod_base = OTHER; note = thymine
  misc_feature 1..23: note = sgRNA sequence
  source 1..23: mol_type = other RNA
ttcatggggaaagcgagaggagg

SEQ ID NO: 50 - RNA, 23 nt, synthetic construct
  modified_base 3: mod_base = OTHER; note = thymine
  modified_base 8..9: mod_base = OTHER; note = thymine
  modified_base 12: mod_base = OTHER; note = thymine
  modified_base 20: mod_base = OTHER; note = thymine
  misc_feature 1..23: note = sgRNA sequence
  source 1..23: mol_type = other RNA
cctggacttgatgcagcagtgga

SEQ ID NO: 51 - RNA, 23 nt, synthetic construct
  modified_base 6: mod_base = OTHER; note = thymine
  modified_base 9..10: mod_base = OTHER; note = thymine
  modified_base 19: mod_base = OTHER; note = thymine
  misc_feature 1..23: note = sgRNA sequence
  source 1..23: mol_type = other RNA
cgagatgcttgcgagaaatgggg

SEQ ID NO: 52 - RNA, 23 nt, synthetic construct
  modified_base 16: mod_base = OTHER; note = thymine
  modified_base 19: mod_base = OTHER; note = thymine
  modified_base 21..22: mod_base = OTHER; note = thymine
  misc_feature 1..23: note = sgRNA sequence
  source 1..23: mol_type = other RNA
ccgacgccggaggcatcatcttg

SEQ ID NO: 53 - RNA, 23 nt, synthetic construct
  modified_base 6: mod_base = OTHER; note = thymine
  modified_base 8: mod_base = OTHER; note = thymine
  modified_base 15..17: mod_base = OTHER; note = thymine
  modified_base 19: mod_base = OTHER; note = thymine
  misc_feature 1..23: note = sgRNA sequence
  source 1..23: mol_type = other RNA
ccccgtctccaacatttctgaga

SEQ ID NO: 54 - RNA, 23 nt, synthetic construct
  modified_base 14: mod_base = OTHER; note = thymine
  modified_base 17: mod_base = OTHER; note = thymine
  misc_feature 1..23: note = sgRNA sequence
  source 1..23: mol_type = other RNA
ccgcgcccggacctggtgaaggg

SEQ ID NO: 55 - DNA, 24 bp, synthetic construct
  misc_feature 1..24: note = Single strand DNA oligonucleotide
  source 1..24: mol_type = other DNA
atgaggatctacggcgaggagcac

SEQ ID NO: 56 - DNA, 24 bp, synthetic construct
  misc_feature 1..24: note = Single strand DNA oligonucleotide
  source 1..24: mol_type = other DNA
atggggctccacgttgatgaacac

SEQ ID NO: 57 - DNA, 21 bp, synthetic construct
  misc_feature 1..21: note = Single strand DNA oligonucleotide
  source 1..21: mol_type = other DNA
atggggattcccggtgacgag

SEQ ID NO: 58 - DNA, 19 bp, synthetic construct
  misc_feature 1..19: note = Single strand DNA oligonucleotide
  source 1..19: mol_type = other DNA
atggcgtgctccttcccgg

SEQ ID NO: 59 - DNA, 24 bp, synthetic construct
  misc_feature 1..24: note = Single strand DNA oligonucleotide
  source 1..24: mol_type = other DNA
gtggcactgaatagggaggagttg

SEQ ID NO: 60 - DNA, 22 bp, synthetic construct
  misc_feature 1..22: note = Single strand DNA oligonucleotide
  source 1..22: mol_type = other DNA
cgatcggctcatcctcaaacag

SEQ ID NO: 61 - DNA, 24 bp, synthetic construct
  misc_feature 1..24: note = Single strand DNA oligonucleotide
  source 1..24: mol_type = other DNA
gagtttcgagccttcctgtaagca

SEQ ID NO: 62 - DNA, 23 bp, synthetic construct
  misc_feature 1..23: note = Single strand DNA oligonucleotide
  source 1..23: mol_type = other DNA
cctgaagtctcgatcgaatctgg

SEQ ID NO: 63 - DNA, 24 bp, synthetic construct
  misc_feature 1..24: note = Single strand DNA oligonucleotide
  source 1..24: mol_type = other DNA
gtggcagcgaatagggaggagctg

SEQ ID NO: 64 - DNA, 27 bp, synthetic construct
  misc_feature 1..27: note = Single strand DNA oligonucleotide
  source 1..27: mol_type = other DNA
gaacggggaagttgacgacgcaattac

SEQ ID NO: 65 - DNA, 23 bp, synthetic construct
  misc_feature 1..23: note = Single strand DNA oligonucleotide
  source 1..23: mol_type = other DNA
gaggcgatcgacatcctgttgcc

SEQ ID NO: 66 - DNA, 25 bp, synthetic construct
  misc_feature 1..25: note = Single strand DNA oligonucleotide
  source 1..25: mol_type = other DNA
ctctatctgatctccgaggttgacc

SEQ ID NO: 67 - DNA, 20 bp, synthetic construct
  misc_feature 1..20: note = Single strand DNA oligonucleotide
  source 1..20: mol_type = other DNA
ggtgcaccacgctcttgtac

SEQ ID NO: 68 - DNA, 27 bp, synthetic construct
  misc_feature 1..27: note = Single strand DNA oligonucleotide
  source 1..27: mol_type = other DNA
atggattcctttccggttatcgacatg

SEQ ID NO: 69 - DNA, 18 bp, synthetic construct
  misc_feature 1..18: note = Single strand DNA oligonucleotide
  source 1..18: mol_type = other DNA
ctcgagctggtcgccgag

SEQ ID NO: 70 - DNA, 20 bp, synthetic construct
  misc_feature 1..20: note = Single strand DNA oligonucleotide
  source 1..20: mol_type = other DNA
accgaagcccctcttaaccc

SEQ ID NO: 71 - DNA, 20 bp, synthetic construct
  misc_feature 1..20: note = Single strand DNA oligonucleotide
  source 1..20: mol_type = other DNA
gtatggctgacaccatcacc

SEQ ID NO: 72 - DNA, 22 bp, synthetic construct
  misc_feature 1..22: note = Single strand DNA oligonucleotide
  source 1..22: mol_type = other DNA
ggggtcatccaaatgggacttg

SEQ ID NO: 73 - DNA, 21 bp, synthetic construct
  misc_feature 1..21: note = Single strand DNA oligonucleotide
  source 1..21: mol_type = other DNA
ggctatatataagtagcaacg

SEQ ID NO: 74 - DNA, 20 bp, synthetic construct
  misc_feature 1..20: note = Single strand DNA oligonucleotide
  source 1..20: mol_type = other DNA
acactccagatagaaagcac